European Patent Application EP 4 151 237 A1, published March 22, 2023. Title: Compounds, method and pharmaceutical composition for modulating Ataxin 3 expression. Applicant: Mitsubishi Tanabe Pharma Corporation. The sequence listing filed with the application follows.

SEQUENCE LISTING (285 sequences)

SEQ ID NO: 1 - DNA, 48070 bp, Homo sapiens
gagaggggcagggggcggagctggagggggtggttcggcgtgggggccgttggctccagacaaataaacatggagtccatcttccacgagaaagtgagtgtccgcgttcggtggggagctgtctgccgcgcggtggcgggcgtggagcgcggcatcaccgcctctcggagggctgggtggggcccgagtcgcccccatgccgatctcgcccggcgaggggcgacgccgcagcctcccgcctcctcggctcgaggaggggagcatcacctacgcccctacttcccccgcggcccccgccctgggagccgggagggagtatgggcggggccgggggcgtctcgggacacgggagtggggtggcgcccagtgggtttgcttctgcctttctccgtcactttccatcgcttttcggaggattccttcacccctccccaatccttccctctccctagggtctagctagagtcatctctgggacacctccctcaacccctcctaccctaatcctggcagaattaacttttcctcctccggactgctcaattctatattggagtcttccctacacgtagatctttggggtcttgttcgtgtctttcccctgcactaggtccgcgagcctcccgagggaggagaccttggctcgcccactgtagggcctgacatttaggaagtgaagtaggaaacccggcgtgcccctaaacagggaagtcgtcacaagagtttttattacgggatgtttgggtttggtttcttttggtactcccatctttccggagcaggcggccagctttgtttttaggtattaggagtggactgggatgattttgttgtagtctgcctagcctgctgtccctttaactcttccgtgaccatgcacttgaagatactgtttgtgatatgtaaagaaactcctcgtttctctcatactattatccagccatttgtgtgtgagtgaagccttccccaggacagctttggcacatggtatcatgtttcataatagtttcgtgtttggaaagagttgctggtaaggctgttatttaataggaggagcaaagggtttttgttttattaaatacttataaatgatcatttatcccagacatttaaaattcacacacacacaacaaataaagcaaagacaaaagaatacatttaccaaatgtaaatctgtagcataaattttttttaatttttattttaaagatggggtctcattctgtcacccaggcaggtgtgcaatggagagatcatggctcactgcagccttgatctcctaggcacaagcgatcctcccgcctctgcctccagagtagctgggactacaggtgcatatcgccagggccaggtaatgtttttgggagagacggggtctcgctgtgttgcccaggctggtctcgaactcctggactcaggtgattctcccacctcggcctctcgaagtgctgtgattacaggcgtgagccactgtgcctggaacaaattgttaagtacaatgcttttcattgtagaaaacatctcggaaacttttgaaataggctgatgttcagtgggggaggaaggactcagtcgtatagttgtcactaattttttgacttgattgacatgactcgtaaatcatagacaatagagatttggttgcttggctgagtagagtgcgtgaaaaatacacacgtacttttttttttttttttttgagatggagtttggctcttgtcacccaggctggagtgcaatggcgccatcatggctcactgcaacctccgcctccccgttcaagcgattctcctgcctcagtctccccagtagctgagattacaggcgcccgccaccacgcccagctaatttttgtatttttagtagagacagggtttcaccatgttggccaggctggtctccaactcctgacaggtggtccgcccgcctcggcctcccaaagtgctgggattacaggcgtgagccaccgcacccggccatatttttgttattaattttcaaaggctttggtgtgggaccacatttcaacatggaaggccttaaacatgttccacactacttcctgagaattagacaagatttttaacaatattgttacctagttgggacacatttgtactgacccatgggatgaaaaaaagctgagtgctagcctagtgaaaatctacttacccgaaagaaatccctcttagtctgggtgcagtggctcacaccagtgctttgggaggcccagacgggcggatcatgaggtcagtagtttgagaccagcctggccaacatggtgaaaccccgtctctactaaaaatacaaaaaattagccaggtgtggtggcaggcgcctgtaatcccaggtactctggaggctgaggcaggagaattgcttgaacccgagaggcagaggttgcagtgagccgagaccgtgccactgcacttcagcctgggcaacagagcgagactccgtctcaaaaaaaagaaaaggaaaaaagagtccctcttaattatcagcatgtgtataggcctacagatacttcaggaatacctttaccattatcatcaacttgtatctacatagcatgtgaagattcaacaatttagttttttgggcgtcctcaagagtacgcacctataaccatatggcccaattgttaatctcctatacagtccattctgggaatgtttgggcttactgtgccatttttccgttcactgccttcccctctgcaatatacctttaacccttgctaggtcctgggtttggagagccagagaaccaactttggccctaaagaagctgtgtaggtagcaatatctgcctacgaagggccttgcaaccatttcctcttggaaccttggtttcctctttctgagtagtcactttgagtaccctttattaagttagaatgtaaaaacagtttctcactgatatatctgcagtgcctgagagagggcctggcacagagtaagtactcaataaatatttgaatggggccgggcgtggtgagacctgtctctacaagaatgaacaaaattagctgggcgtgttagcacatgcctgtagacttgggaggctgaggtgggaggattgcatgagtctgggaggtcgaggctgtagtgagccatgatcgcaccactgcactccagcctaggggacagagcaagatcctgtctcaaaagaaaaaaatgtatatatttgaatggataaagagatggctttgagtttctgagatatatatggtgctgtttatctaaagtaaacaagttttctgtaaatattttaaggctttgcaggccagctgtagtctctgtcacacattcttatttgtgcatgtttttcccaaccatgtaaaaatgtaaagtgcattcttagctactggggcaggttgaatttggcccatgggctagagtttgccaacccctaacttaaacctttgtactaactttatgaccactactggatttttgttgttgtttgttttagttctggtgcctgctttgtttttttttttttttttaatcctcttgctgatgtttcttggtgcagttactgtgccatttgtattggtgcttttaatgtaatgcaaactggtaataatatctaaacttgctggggttgtacataaaattattgaaaagattgaaaagatgctgagcattgactctgtggcattcattatgcccttttgtgattgctggattttagccatctttaggacatttgagctttaggagaagccaaattctgtataaatgacttgaagtgctaatagcacaggttttgaaacctctgcctgggtttgagtctcagctctgccttttactacctgtgtgatcctgagcaagttacttagtatccctgtcctctagtttcctcctctgtagtgtggggataataacatagacataacctgagagttagagtgtagagaaggctccctggcagatagtgctgtagaagtactggccattgccattactcaggtgcttgtgtttgctgaacctcatagtaagggctcggagagcactaagaggaggtgagaaatgctgctagattgacagcttgtccccagatagcccattcccgagagcaccttaggtttatacctgatttgtgttgtagttagtagtgtctctggtaatttgaactagtttcaggttggtcttgaaaacctggggaggttgggggtaaatgatttggtagcagttctcttttgtgattttatacattatctttgtagaactgcagtttgctaattctctgagcccaacacaatgaagtctgggcctaaaatcatagaatttcttttatttttttttttgtttttaatttatttattccctccctccctcctttcttcctttcttccttttctttctttctttccttccttccttccttctttcttttctttctttcttttctttctttggagtctcactctgtcaccaggctggagtgcagtggcacgaactttcttcagagtctcactttgtcaccaggctggagtgcagtggcgcgaactcagctcactgcaacctccgtctcctgagttcaagagattctcctgcctcagcctcccgagtagctgggactataggcatgtgccaccatgcccagctaattttcttatttttagtagagacgaggtttcaccatgttggccaggatggtcttgatctcttgacctcgtgatccacctgcctcagcctcccaaagtgcggggattacaggcgtgagctaccacgcccagcctattttttattttttgaggcagagtctcactctgtcacccaggctggagtgcagtggtgcaatctcagctcactgcaacctccgcctcctgggttcaggtgattctcctgccttagcctcctgagcacctgggactacaggcgcctgccaccacacctggctaattcttatatttttagtagaggcggggtttcaccatgttggccaggctggtctcgaactcctgatctcaagtgatcaacctgccttggcctcccaaagtgctggaattacagccatgagccaccatgcccagccaaatcatgagatttcaataccgctgaactttgattatggcaaagtgaacttctgctttgattaaagcttgatgagagaggtggctggggatagtttgagataagggcaaggcaggaaaatgcataatcttacgtgggctcattgtcattgtacaattcttttggtccatgtggaatttgatccgtcctatgacttaagttatgtttatttttgtttttatttttatttattttgtgtctttttgagagacatgatgttgctctgtcacctgggccagaatacagtggcacaatcttagctccgtgtagccttgaactcctgggctcaagtgatcctcccacctcagcccctcaaacagttgagattatagtatgaaccactgtgcctagccttaagtgatttttaaatttgtactgaacagtttgtcctttccttccattaaatcatattagaagtacagaacttgatatttcctgtagcaatacagtttttctttgatgaagtttgatttcaagtacttatttttcataatttaaagctattttttatagagagaattttaatcaaatatttggatgtcactattgctatatatggtattaagtatggtgaccatagtttgtaaactccaaactgacagcaagacaggaaatttgtgttagcaaaggcttttttcttactgtttgaattttttaaaaattagatacaatacagagaggagcacacaaatcattaagagtacagctcagcgaattttcacacagtgaacatgtgtaaacagcaagtaacaaaagatttacctgcatcctataacctcccattattcccttttctaggtactgtctctccactgcattcccaccaaatataaccactatgctgaattctgacatcataaatgagttttgcctgattttgagcttttgtgactggaagtgtacagtgtatataccctttcgattctgtcctctttagtttaccattgtttgagaaatttatccatactgttccagaattaactactgttaattattgttaattaactactgttgtagttaattcatcctcattgttatctagtattcttttgtgagtaaacacaatttccattctactgtgatcccagctatccatttgggtcgtttccagtttggggtccattacaaatagtaatgctatctgtaatgctattttgtattactacaaatagtaatgctatttgtggcacaaaaatactgcttttgtgaacattcttatacatgtcttttgatgaatgtatgtttgcattgctgttgtttacattatgtacctagtaatggaattgctagatcataggagatgtatatattaagctttagtggatgcattacataattattagttattattggttataccaatttatcctctcatcagtagtatacaacagtttctgtatctctaatctccaacattttagccattttagagtttgtgtactaacacattgtggttttaatttacatttccctgatgactaataaagttgagtacctcttttgtgttctttatagccatttgactgtcttgtgaagtgcttgtttgtcttgcctatttttcttttctttctttctttttcttccttccttcctttctttctttcttctttctttccttccttcttttctttctttctgtctttctttcttgtctttcttgtctttctgtctttcttggtcttgccctgtcacccatgctggagtgcagtggtgcagtctcagcttactgtagcctcgacctttttggggctcaagttatcctcctttctcagcctcccaagaagctggactacaagcacgcaccaccatgctcagttaattttttattttttgtagaaatggggtttcaccatgttgtccaggctggtctcaaacttctgggctcaagtaatcctcctgccttggcctcccaaaatgctgggattacaggcatgagccaccgcagccagccttggctatttttcaaaaggatataagtagaacatctgtatatcccttcaatttgcatattattcagtaagagttgcactctggtagtagaaatatataaggaggagaaagaagtggaaacaaaaagtctattctcatgagaagacttgggggatagtgttctctctagctccaagctacttattccttacgaaaagttgaagataaacttatctcagactgaggctgtctcaatgttgtcttcctattccattatacacatataacccatatttttttcaccagctgaattttgctcctagaaaattgattcatcaggaaaaatatccgtcttgcaaggtggttctctttagagtctgctgtgtgacatagctcaggacaaattgtgtgatgtcagataggttgggttaaggaatagaccttattggggaaagagagaacttggagggccaaggttagcaggagaaggaaatgttctctcatctgccgtcaattcagggaggggcaaacctggtgtctgtgttcacagggagggatccatccatctgtgattctcccttcttatcaggtagcatgggaaagctacactgttgcggggaggagggtcacacgcaggctacttagtaccaggcaccctggacttggattcaggttgccagttgtgtgagaaactgcccagcacctgaaggccctgaacccatgagaagttgtacctacctcccatgaggaggaatcctgtcatcccatgggagctgagcttgggtgcagtccctcttgctggcttgtccaggagtgagctccagggttgtttgggacagttctgctcattgctttacactgtgtatacattatctgtagagttccatgaagagaacttcagcactgtaactgcaagttttaacatggaacagaatttttctcacctgtattaattcttaagatttgaagttctatcaacaagcatttagattgtgtggagatttttttatttttatttttggagacagagtcttgctctgttacccagactggagtggcagtggcatggtcttggctcactgcaggctctacttcctgggttcaagcgattctcatgcctcagtgtcctgattagctaggactacaggtacacaccaccatgctggctaatttttgtatttttagtagagacgaggtttcaccgtattggtcaggctggtctcgaactcccagcctcaagcagtccacccacctcggcctcccaaactgctgggattacaggtgtgagccaccatgcttgactgacatcatcatgttaaaagaataaatgttctagggagctgggcacagtgtcatgtttctgtagttctagctgctcgggaggctgaggcaggaagatcccttgagccctggagttcaagtccagcctgggcaacatagtgagatctctttttttaaataaataaataactgttctagggactaaaatttcctttcaccattagtaatttactgtagaatctccaagaatgaacttattttaggtactgaaaatgagggagactaaatgttttatacagtagtttttagtaaaatatgagatttgatgcatttgatagatgatgtttgtttaaaataattcttaaatttttgatcatgtaattatagtttcattaatggtagatttgtaaaataaatgttaccaaatgaaaatgcatgtacctatgttaattatccttatctaaagctgaaagttcagttcaactatgttaaaacatagtaggggcctggcagggtggctcttgcctgtaatcccagaacttagggaggccaaggtgggcagatcacgaggtcaggagatcgagaccatcctggctaacattgtgaaaccgtatcgctactaaaaatacaaaaaattagccgggcatggcggtgggcacctgtagtcgcagctacttggtaggctgaggcaggagaatggcgtgaactcaggaggcagagcttacagtgagccgagatcatgccactgcactccaggctgggtgacagagcaagactccatctcaaaaaaaaaaaaaaagttggccaggtgtggcggctcacacctgtaatcccagcacttttggaggccgaggcaggcggatcacaagatcaggagtttgagaccagcctggctaacagagtgaaaccctgtatatactaaaaatacaaaaattagccaggcatggtggtgcatgcctgtagtcccagctacttgagaggctgaggcaggagaatcacttgaacccgggaggcggaggttgtggtaagctgagattgctccactgcactccagcctggacaacagagcaagactctgtctcaaaaaaaaaaaaaattaatgattaaattatttaggggagccgggcgcagtggctcacgcctgtaatcccagcactttgggaggccaaggcgggcggatcacgaggtcaggagatcaagaccatcctggctaacacaggatgaaaccccgtctctactaaaaatacaaaaatttagccgggcgtggtggcgggtgcctgtagtaccagctactcgggaggctgaggcaggagaatggcatgaacccgggtggcggagcttgcagtgagccaagatagcgccactgcactccggcctgggtgaaagagtgagactccgtctcaaaaaaaaaaaaaaattatttaggggaagatactatacaattctgtttaacaagtcacattttaattttttcttttggaaatattagcaagaaggctcactttgtgctcaacattgcctgaataacttattgcaaggagaatattttagccctgtggaattatcctcaattgcacatcagctggatgaggaggagaggatgagaatggcagaaggaggagttactagtgaagattatcgcacgtttttacaggtactgattttaaactcactaagtcacatttcttttttttttttttttttgagacggagtctcgccctgttgcccatgctggagtgcaatggcgcgatctcggctcactgcaacctctgcctcccgggttcaagcgattctcctgcctcagcctcccaagtagctgggattacaggcacacggcactatgcccggctaattttttgtatctttgttagagatggggtttcaccatgttggtcaggttggtctcaaactcctgaccttatgatccacctgtcttggcctcccaaagtgctgggattataggtgtgagccaccacacccggcttacatttcttttaaaaatgtggataccatttagaaaaggatgggccattcttcctatagggatctgactggtgaattataactgtgctgttaactttggaaatgggaatgcacaagatattgttttaaatatgcacgctaatgacagtttgtatccttctttccccacccccacccttgcttcaactacctgtcaaaattaacagcagccttctggaaatatggatgacagtggttttttctctattcaggtaagtagtcacaagcatgtactatgtgttgcttacatcccaggcaccgtttcacagcctttcaatagtcactgtaacaaggcgaccttcggaagttcttctgtctacagagtatagattatactctagagtactagattttttttttcttgagacagagtctcgttctgtcacctaggctggagtgcagtggcgtgatcttggctcactgtagcctctgcctcccgggttcaagcgatcctcctgcctcagcctcccaagtagctgggattacaggcacccgccaccacaccagttaatatttgtatttttagtagagatagtggggtttcaccgtgttggccagtctggtctccaactcctgacctcagcctcccaaagtgctgggattacaggtgtgagccactgcacctggccaactagagtactagatttttatatagataaacatgaaaggattgtagaatcttcatattagagtggggcatttaaaaattccttcttgagaaagattaatttgcatctggatgctaataataaccttaattctggccgggcgcggtggctcacacctgtaatcccagcactttggggaggccgaggtgggcggatcacgaggtcaggagattgagaccatcctggctaacatggtgaaaccccgtctctactaaaaatacaaaaattagctggacgtggtgacacgtgcctgtaatcccagctactcgggaggctgaggcaggagaatcgcttgaaccagggagtcgtaggttgcagtgagccaagatcgcgccactgcactctagcctggtgacagagcgagactccatctcaaagaaaaaaagaaatccttaattctaataagtcacaatgtctcaaacttaccatctgttgggtaaatttgagaaaatgcaataccttgctaccatccttttaaatcagcctaccagactggatttccttattatggtttgtggcttttgattttttttttttaatgtatagctctctttgaattctttggtggttatatatatatgtactcgcaagattcttttatctgtgggtctttcattctttttctaacactgtgagttgtatccagagtactttcggaacctctcctgagcgacctatctctgcagatatctttgtttatgtttcccttgtactgccctcctggactcttcctcatccaccagcatttccatctagtgctttaccgtgccactgctaacaggtaatggctactgcagggctgaaatcagaggccagagtaggcccagcacttggcgtttcctatttgtgccttgctgctcttggtgcctgttcatgtgtgcccactaccttgcactcaatttctgtctttgctggtacctggctcacttgcttctttgttggctaccttggagggcagatagtgaattttcagaaatttccctttttttgtcagacagattgaaataaacaggtttgcattttgttttttctacaagcggcaagcccatgaccctagaagtctgacatctatggaaccttcagtttaaatgcccagggagaacttattttggtagatatgatttctgacattgcaggtagcaagttgaatataatttttctaaagtagcacccacagcagccaaattatcagatgtatatagtagactagttttaagaaaagcacttatgggtagaatatacatctggatttttgaggcagttttatttaggaattgtgtggttttctggaacatctcagagacctggtatgaaaagcactcttctaatatatatgtgtttttttttatggatttagtgatatatctatacacacacactttttaaaacctatagccggctgggcgtggtggctcatgcctgtaatcccagtactttgggaggcccaggcgggtggatcacaaggtcaggagattgagaccagcctggccaacaaggtgaaaccctgtctctactaaaaatacaaaaatagctgggtgtggtggcgtgtgcttgtaatcccagctactcgggagcctcaggaggagaatcgcttgaacctgggaggcggaggttgcagcgagccgagatcgtgccactatactccagcctgggcgacagagcaagactctgtcacaaaaaaaaaaaaaaaaacctatagccttctagagaaatttatatatgaagtacacaactaacatagctacacttcctaaatttggaatggagtggtttagcttatgaaaagttgctatttttcttaacaggttataagcaatgccttgaaagtttggggtttagaactaatcctgttcaacagtccagagtatcagaggctcaggatcgatcctatgtaagattctgttttgcatttcatacatttcttttcccaaatttgatttttaaagttgtaatttcttaaagaagagaaatacattttgaatacttttgttttgatgttccctgtttcattcactcagactttcctatttcacctttgtgatgtccatgagcatctgccctgtagccttcctggcaccccagtgtctgtggcagcacagagctgaccccataagtggtgcatgaggccatcttgtggcacagcatcactaagctgctgcagagacgttcatatggttgtgtgatcttttaaaaacatcagtgacacttaactataaatataatcttaaattatcacaaattttatataatatttgccagtagacaacataaatatgaattcaatatttcaagttaatattgtctgttttcttttttagaaatgaaagatcatttatatgcaattataaggaacactggtttacagttagaaaattaggaaaacaggtaacatttcttacccttccttgtctttttttcttatattgtaccccatttaaaactaaaatgtgggccaggtgtggtggctcatgccaacagtttgggaggctgaggtggggggatcacttgaagccaggagtttgagaccagcctgggcaacaaagggaggtcctgtctcttaaaaaaaaaataaaaataaaaataaaaataaataaaaaaaaaaacaaagagccaggcatggtggctcacatctgtaattccagcttacttggaaggctgagtcagaaggatcacttgagctcaggagtttgaggctgcagtgaactatgattttgtcactgtaccccagcctgggtgacagagtaagactgttctataaaacataaaaataaaaaaaatatatttaaaaattaaaaaaaaaaaaggattgctgactttaaaattaggaaactgaccagtaatgtgtgtgtgtgtagcatggtttatccttcttgatagatagaaattgtcattttaaaagataatatcagttttccttataaatttatttgtgacaagtatatgcaatttaactatatcataagaaaaattctatattaaagataatacaaatgtggttacttttaagtgggtttttatgtgatgactatgttctgtcagttaattattacatttatagatttgtatttagcatagtgctgtcacaaagcctgaaatagtgtcaagcatgaataaagcattcaattatgtttgctttagtgtaagattattcattatgattccaaaagccatgtaatacgtacgtctacagaaaatcacttctattttttaaataaaacatgaaatatgtcttgagcaagctattttaagaaacaatcatttaacgtccttgttattagaattttgaatctttgaaagagggttattgaaaaccagctaggacagtaaaaaagaataaactagtgatacatgcagcaatatggatgaatctcaaaataattatgctgaaagaataacccacaaacaaaatactacctgctgtatggtatcatttattaaaagtctagaaaagtgcagattcatctgtagtgatggaaagcagattgaccagcggttgcctggggacgagaaggctatggaggagtgagaggggagggttacagagaggcacgggaaacatggcaatgaggaatgtgttcactatcttggttgtagtaatggtttcatgggagtacagtatacaaatgtgaaaacatttcagaggccagatgcagtggctcatgcctgtaatcccagcacttttggaggccaaggcaggaggattgcttgagctcaaggagttcaggaccagcctgggcaatggcacaagaccccatctctaaaaaaaaaatgaaagaaaaaaaaattggctaggcgtggtgatgcatggccgtagtcccaggtgctagggaggctgaggagggagcacagaggtcaagcctgcagtgaatcatgatcgtgctactgcactccagcttgggtgacagaaggagatcctgtctcaaaaaaaaagtttcaaattatacactttaaatatgtgcagtttattatatgtcacttataccccaataaatctgttttttttaaaatgtaaatacaagccaaaaaaggtataagtcaagaaaatatattgaattaaatctgtaagagataattcaaaaacaaaaaccctattgttatcttttaagtcacccaaatcaaatttgggaaaagtcacctacttagcttcatcctaagttggttctttctttctttctttccttcttttgagacggattcttgctctatcgcccaggctggattgcagtggcgggatcttggctccctgcaacctccgccacctgggttcaagcaattctcttgtctcagcctcccaaatagctgtgtctacagccacgcaccaccacacccagctaatttttgtatttttagtagagacggggtttcgccatgttggtcaggctggtcttgaactcctgacctcaggtgatccgtccgtctctgcctctcaaagtgctggggttacaggcgtgagccaccatgccgagccctaagttggttctttcttaaagttcttcctgaggagccaagagcaagttaaggagatgtaacctagaagcttacagtggaggctagctgggtgcagtggttcacgcctgtaatcccagcactttaggaggctgaggcagggagatcactgaggccaggagcttgagagcagcttggcccaacacagtgacaccttgtctctacaaaaaaaaaaaaaaaaaaaggcagcttacagcagtagaggctgatgcgagtgggaatcacctctaggtaaaaaccagtgtagcgtactgctgagattatttaacctctgggttttatttatgtgtttttaaaaattatgatccagtattttttacttttttttgtataaagtaagcactgaatttttaaggttgtattaatttgcaaataaatgtctatcttattattttgagagatttaaaaaattttagttcttcaaaattgcattttcacattttgaattacgttatctttgacaaatacagaagatgtcaaattttggtttattttctttggttctaatttatatttttgtttaaaactatatttttcactatagactctttctgtctctcgaggtccctgtataatgaaaaagaaggctggaaaaagtattaacattgtcaaaatccaggaaaagtagttggtcatgatattgatcgttaactttagaaactttttgtatcttgtgggttaaattaggattactatgtggtagtgataaatgatgttaattagggccgagtgcagtggctaacacctgtaattccagcatgtagggaggctgaggtgggaggatgtcttgaatccaggagtttgagaccagcctgtacaacatagtgtaagaccccttctccacacaaaaaaattagaaaatttgtcaagcatcttggtgcacacctgtagtcccagctgcttgggaggatgaagcgagagaatcacttaagcccaggtgttcgaggctgcagtgagctatgattgcaccactgcactccagactagatgaccatctcttttaaaaaaatgtgtttatatgttatatgtgatagtgctttttaaaaacatttttaaattatagagacagggtctcactatgttacagcccaggctggtctcaaattcctgggctcaagcaatcctcccaccttagctaacctcccaaagtgctcggattataggcatgagctgcatgcccagctaatttagtgatttttaaaaactgagctggtaattataaattctcttcctggaacttctgactttctcacaattggaatcttttgacaaaaattatcagtaatgggaaaactttgtgtagttgtcatttttcctcccatcagtgtgatagatatgattggagttatgttggactgatattttgaaaaaagatttaattatagctattaataaagacatttaaactactgactatgcatttttattcttttgggagggtttaatgtttatagtttaaagcaaactgttgtttttaaaaaagtatctaacagggccgggcgcggtggctcacacctgtaatcccagcactttgggaggcctaggcgggcggatcacaaggtcaagagatcaagaccatcctggctaacatggtgaaaccctgtctctactaaaaatacaaaaaaatagctgggtgtggcggcgtgcgcctgtagtcccagctactcgggaggctgaggcaggaggatggcatgaacccgggaggcggagcttgcagtgagccgagatcgcgccactgcactccagcctgggcgacagagcaatactctgtctaaaaaaaaaaaaaaaaaaaaaaaaagagtatttagcagaggccaggtgcagtggctcatgtttgtaatcccagaactttgggaggctgaggcgggcggatcatttgaggtcaggagtttgagaccagcctggccaatgtggcaaatgtgctgtctctaactaaaaatacaaaaattagctgggtgtggtggtgcagacctgtagtcccagctacttgggaggctgaggcaggagaatcacttgaacctgggaggcagaggttgcagtgatccgagatcatgccactgcactccagcctgggttacagagtgagactcttctcaaaaaaaaaaaaaagtatttaatagtgataaatctgcagtattctcttgtagtttttaagatcatattattcagtcaaagaaaagagctcaacttgaaatatttccagagtttaaacaatcttactaagctttgatgggttgtatctattcttaacatgtgaaacttccttattacctataatatacactaacttaaatattgacaatttttttccagtggtttaacttgaattctctcttgacgggtccagaattaatatcagatacatatcttgcacttttcttggctcaattacaacaggaaggtaagtaacggctgaacattttgtaatgttacctttcgaagtagttaaataaccaggcacattagatgacagtgtgataaaactgtttttctggcagtggcagtgaaacaatctttagttttgacgtggtgataggctgtgatttgggtgacgctgttcagttagagttctcactgacacctggcccttcctcttctgaggatgctgctttctttgcagcccttctaagtaatggctttttcttttatacatcacatatcacacggctgagaggagggatagatgtttttcttctttgcctcttctaggccactgttcttccttataaactccagtttctttgaaatacatgcccctaacggctgggcacggtggctcacgcctgtaatcccagcactttgggaggctgaggcaggcggatcacgatgtcaggagatcgagaccatcctggctaacacggtgaaatcctgtctctactaaaaataacaaaaaattagccggggtgtggtggcggacgcctgtagtccgagctactcgggaggctgaggcaggagaatggcgtgaacccaggaggcggagcttgcagtgagctgagatcgcgccactgccctccagcctgggcgacagagcgagactccgtctcaaaaaaaaaaagaaaagaaaaaaaaaagaaatacatgcccctagattaaactatcccttgtccttttgcactcatccacaagtctcttttcatcagtgattttaggatctgactcgttgtctttttctctacttcaactacttttatcattcttaattatttctgtatcgtcaatcaatccagtacctgcctcttagtttcaaaatcacttactcttgcttagctattaccagtaatcataaccactgtcaaatctcaattgcaagcatattactctttaactaccacctcctatctttaaaccatgttttgtctgtttttttattccagccattctttaaaccctactgtggggcccaagcatttcctttatacgcattcttcctttcttctactgcttattttctgtaatccgtcatcataatcactccattgcattcttcaacgtgtttcccctctctccctccatcatacttgaatgacaaaaatctcaaccctggttaaaccacatcttggccttgtccattcctgtaccagagtagctggacgtggctaaaaaataacataaaacatgatgattggttttacttttttcttaaatgatctatccatccattcacccatccatctatcaaagtgactaggcctatttctgaagcccaggctggagtgcagcagcataatcacagctcattgcagctccaaactcctgggctcaagtgattctcttgccttagcctgttgagtagctgggactacaggcttgtgctaccacacctagctaaggttttactttaaatttattataatcacaaaattcagatgagcctttagtgctgtctgatatttctactatgttttcttagtgatgtaccaccctccaaggtgtttataaaaaattatgtaccactctccaagaagtttataaaaaataatgtgccaccctccaaggtgactaatttcacagcttatgtctttaaacctttaagcactttcctctcccttacacaccttccttgtggctttccgttacattctgctgagaacatagaagcaattaaaattatgttctttctaccagcaaatttatcaatttgcttatatcttcacctgtgctttgagcctatttaaatagatgaatggtcccctacctctaaccaaaaccagtccctcacttgtgggctggatcccagctcttctcacctactcaagatgttcctgctttcatctctccactctcttatataatcagttccccccccctttttttgtaatattcctataagcagtaaaataagctttttatttccattgattaaaaataaaaatcctctcttaattccatgaaactccagctgcctccccatttttattttttccttaggattgtctctagtgtgccttctccttttcttgaactctgcctcctgggttcaagcgattctcctgcctcaacctcccgagtagctgggattacaggcgtgcaccaccatgaccggctaattttttttttttttttttgagatggagtttccctcttgttgctccggctggagtgcaatggcgtgatctcggctcaccgtaacttctgcctcctgggttcaagcgattttcttgcctcagcctcccgagtagctggatttacaggcatgtgccaccatgcctggctaattttgtattttagtagagatggaaggggtttctccatgtttgttaggctggtctccaactcctgacctcaggtgagccgcccacctcggccccctaaagtgctgggattacaggcatgagccactgcgcctggccccggctaaattttttttttttttttttgtatttttagtagagacagggtttcaccatattggccaggttggtctcgaattcctggcctcgagtgatccacctgcctcagcctcccaaagtgctgggattacaggcgtgagtcaccttgcctagccatcttttagtaatggtatttggagatcacaatttgagtgctggcatgcttattgctgctgggtttgttatgtagttattgtgaattcacatttaggaatatagggtttttaattctttgattttagatacttgtatcttttttcttttatatttaaaaccttggttcctgatgatatcccttcttagaaaccctgtctacctttggccttcagcccaccatgctgtggttttcctaacttgctgcctgcacttttcagattcctttcatggatcttaaatatcatctgtaaataagatctatgtgtcaataattaccaaacttttatctttagtcttgacatctaccctgaacacctagctttgactaactcctagctttggcatctccacttggaaatccaaaaagtgtttcaaactgaacatgtctatgaaagacttatttttttctctctatccatgctatccatcaggttttccatttccataagggtgactcttgtactctggttcctatatattataccgacagagcagcccagagtgcttcttaaccagtgtaaggcctgttatgtcccaccctcactctttgtccttcagtggcttcccagcacacttagaataaaatctgaagtcttaggccgggcttggtggctcatgcctgcaatcccagcactttgggaggatgagggggcagatcacttgaggtcaggagttgatgagaccagcctggccaacatggtgaaaccctgtctctaccaaaaaatacaaaaattaactgggtgtggtgttgtgcacctgtagtcccagctactcgggaggctgagataggagaatcacttgaacccgggaggcagaggttacagcgagccaagatcataccactgcactccagcctgggtgacagaacgagactctcaaaaaaaaattaaaaaaaaaaaatatgtgaagtcttgaataaaacccaagatctttaccatggcccctgaacagggcagagtatccattcttcagacactcttcatagaataccatggtgagctggcatatttattatacaatacagaaacaattttactggcagaaaacacattaaaccgtctaaactctgaatacagttgtcctcataaaaaatgttcaacatactattttgaggttttccattaatagttcttataatctttgtcccattatgtgttaatccaacaaaggatatccaataacaaacaccaaagtttaagaaaaatgtgctaggcgcggtggctcacacctgtaatcccagcactttgggaggccgaggtgggcagatcacctgaggtcaggagttcgagaccagcccagccaacatggtgaaaccctgcctctcctaaaaatacaaacattaactgggtgtggtggtgggtgcctgtaatcccagctactcaggaggctgaggcaggagaatcgcttgaacctcctgggaggcagaggttgcagtgagctaatattgcaccactgcactccagcctgggtgacagagtgagactccatctcaaattaaaaaaaaaaaaaaattaatgatagagaaacttaaatcagttagattgttttaggtatagcccatccttggtttttgtgtgtagcatctagcttggggaaaccctggatttctggaatcatatttagacacagtcacactagactaatgtaattcttttgggatgcaaaccacacgtttgacaccttaaatagcttttaggtatttggcttcccagcccctatttttagttacaaggggtgtacatgtgtgggtcagggtgggggtagctctttccgcagatgattagttttagccatgttactagttattgcacacattatctgtgtcctcacagcagccctgtgagtaagtgtattagggttctctagagggacagaactaataaggtagatgtatatatgaagggtaatgtattaaggagtatcgactcgtatgatcacaaggtgaagtcccacaataggctctctgcaggctgaggaaccaggaagccagtccaagtcccaaaacctcaaaagtagggaagctgacagtgcagccttcagtctgtggcaaaaggcctgagagcccctggcaaaccactggtgtaagttcaagagtccaaaagatgaagaacttggagtctgatgtttgagggcaggaagcatccagcatgggagaaagatgaaggctcagcaagtctagtacttccacactcttatttctgcctgctttattctagctgagctggcagctgattagatggtgaccacccagtttgagggtgggtctacctctcccagttcactggcttaaatgttaatctcctttggcaacaccctcgcagacacacccagaaacaataatttgtagccttcaatccaatcaagttgataatattaaccatcacaggaaggtactagtatcatatgtttaacagtagaaaccaagacaaatgcagctaggaagtgggagaactgggatcagatgcaggcagtctgattctaaatcagttgctgttacccactctgacaacagtaagtgagtagcctgctcagtcaagtactatattagtagggccctttacagacatatttatttctcacagtcactcaatgagacggctcttccagtcttacaatggagaaagtgaggctcagagactttaagtaacttaccttagacgactttactagtaagtataagaatcattatttggactaaagtctttctgaatcctcagcttgtatttttttccagtgttctgtgctgcctttttatctactagtgttttacatcaattttgaatctctttactaactggttaggttgatttttgccttttttttttaggttattctatatttgtcgttaagggtgatctgccagattgcgaagctgaccaactcctgcagatgattagggtccaacagatgcatcgaccaaaacttattggagaagaattagcacaactaaaagagcaaaggtaaaaatgaggcctgcagtatggaatatatggtagtatttcattatgagaattaaattttcatgcttagattgaatatgtggtccttgtgttgttggcgactctattttggaccttatattttagtgaagtttattagtttaaacttgaatcaactctttgaaatacttaaatatattaacttagttagctggtatggtatattcctagcacttcgggaggctgaggcaggctgattgcttcaacccaggagttcgagaccagcctgggcaacatggcaaaacctcatctctacaaatagtacaaaaattagccagatgtggtggtgtatgcctatagtcccagctacttgggaggcagaggaagaaggatcacctgaaactggggaggtagagactacagtgagccataatcacactaccgcactccagcctggtcgagagagtcagaccctgtctcaaaaaaaaaaaaaaaaagaaacggaaaaaaaaaacttagttggattcaaattgcaacacaatcattatattactagagcttatttgccagaaaacattttaagttttgacttacttaaagcctttacattacaaatgcctttatgttatgtctaaaatagaagattggttgcagttattaccagtgcttttgttctttagagtccataaaacagacctggaacgagtgttagaagcaaatgatggctcaggaatgttagacgaagatgaggaggatttgcagagggctctggcactaagtcgccaagaaattgacatggaagatgaggaagcagatctccgcagggctattcagctaagtatgcaaggtaaagacattctgatgtgtgttgtattcattgctgaagaattgattccaattattcttagatttcatggaagttaatgtactcttagaggtgttttgacaattactgcagaagcaatagctatatagtgggctttccctttagatttcttataatggaaatcactttttacaacctatattttattaggagtagttatatttttactcctggttattttatttggtttcaacactgtactaacacaatagtaaattgtggttttaatctttgtgggtatcagttgacccttatccaaatcagctgttacataaatatgtgccattagacactatggaagggcctggacagggaatataaactgattttacaaaaacccaacatttattggctatgcaacttaaaccgtaagcccactttggtgggcccagttttttagtgatataaactatcaatagagaaaagcgaaaacatatcccctagacaatctaggcaaagaaaaatgttaagacatagctcaaagtagcttaattaaaagtttgaagtgggttttttgttttatttttttctaactcatatgtatttgcttctactttctaatgaaattatttatcagttgatttccttagatatctaaataaaattgaaatttcattaatgggaagattatttttatcctgaacttttcttgcctctatgcatgcctctgagtactccatatggtgtgcaatcccatttttgattaatagagtcctgctggattagcagggacagaaatcagctttagatttctttcttttttttttttctttctttttttttttttttttttttgagtcagagtctcactgtcgcccagcctggagtgcagtgatcttggctcactgcaacccctgcctccgaggttcaagcgattctcctgcctcagcctcctgagtagctgggactacaggcgcctaccaccacgcccagctaattttttgtacttttagtagagatagggttttgcccttttggccaggctggtcttgaactcctgacctcaggtgatccacctgccttggcctcccaaagtgctgggattacatgtgtgagccaccacgcccagccagaagagtagaatattcttaaagagaaaacgttttaaaggcttactcaaatgagtataaacaaacatattgttgcttgaattggtaaatacagtgattggtttttgttgtgttgtgttttgttttcaggtagttccagaaacatatctcaagatatgacacagacatcaggtacaaatcttacttcagaagagcttcggaagagacgagaagcctactttgaaaagtaaagtagttggtacaagttaaagtagcatgtttaatatttgctttggctattttgtctatttgtaaatggttactgcctgaatcctgtgaatatttgaatgtattttttaaaaatttacagcaaataggacgggcacggtggcttacgcctgtgatgctagcagtttgggaggccaaggcgggcagattgcctgaggtcaggagttcgagaccagcctgggcaacacagtgaaaccccatctctactaaaaatacaaaagaatcagctgggcatggaagcgtgcgcctgtagtcccagctgcttgggaggctgagccaggagaattgcttgaacccgggacgtggaggttgcagtgagccgagatcgcaccactgccctccagactgggtgacagagtgagactccgtctccaaaaatatatgtatatatatataaataaaaataaaaatttacggcaaataacatgaaacaaaaaaaccttgccccaatactggataaattttttaaactgagtgaaggaaaccttataaaatttcatttattaaaagaaaaatgaaattaggacaagacaagaagaatgccaattgatcctttggatgtacttcttgcttacctgattaaccctgcaaaattcctctaccaatcagtacgaaaaacagctttggaggtatgggagcgcattcccaaatagacgtggtagttcatttagctgctcatggccgcttcaggcagtcctgtaagcctgttagcatcaggggaatggatgcaaaccataaatctggatcaactcctaaaaccttaccttgtgcccagccttgtaagtgcttgctaaataggaattccaccatatgaaaatacattcttttcaagtaactatcattcagacttttgtcccccactttttttttttaaagaaaaataaaaggctgggcacggtggcttacgtctgtaatcccaccattttaggaggccaaggcaggtggatcacctgaggtcaggaattcaagaccagcctgaccaacatggtgaaacctcatctctactaaaaatacaaaaattagccgggcatggtggtgggtgcctgtaatcccagctacttgggaggctcagacaggagaatcgcttgaatctgggaggcagaagttgcagtgagctgagataacgccattgcactccagcctgggggacaagagcgagacttcgtctcaaaaaaaaagagaaagaaaacttcatgttaaagattacaagataaataatcagacccactgatcctaggtcagaaaacagagtcatagctcaatctgacttactatttgctgtatttcatccattctgagatgcacatagtttcacatttcaatgtctctgaaattgagaagcatcttacagtcataattgacagtatattagcagcacctataaatattggctcattttacatttgatggtataatgaagaaaatatttacctttttttctgttttgtttttaagtcacaactcagaagtagatgaaggaaaattctgatcagctgacatcctcttaatgtgagatatttctagtctttattcagtatagattaatggctaattatatgttaaatttcaaagtagtgcttattagtgctttttacttttaagtttcaaaattaacttttttattataataaactccaaatttatacaaaagtagaaaaactagcatactcctgtttatgacccagattcaacaaatactagcacacggccaatcttgcttttttttttttttttttttgagatggagtcttgctctgttgcccaggctggagtgcaatggcacaatttctgctcactgcaacctctgcctcctgagttcaagcgattctcccacttcagcctcccaagtagctgggattacaggtacacaccaccatgcctggctaattcttgtatttttagtagacacgggatttcaccatgtcgtccaggctggccttaaactcctgacctcaagtgatccacctgcctcggcctcccagagtgctgggattacaggcatgagccactgagcccggcccaatctcgttttataatactcccatctcccattctttccactgtcccacctgcaagtttggattattttgtaacaaatctcaatcatcatattattctataaccattttaatatgtgtctctaaaatatattagctttatttttaacatagttaaatgctattgtcataaaataataatcataataattaattgtaattctatatcatcaattatctagttaatgtaaaaaataaatctaaggccaggcgcggtggctcacacctgtaatcccagcactttgggaggctgaggtgggcagatcacctgagatcaggagttcaagaccagcctgaccaacatggagaaaccccatctctactaaaaatacaaaaaattagccaggcgtggtggcgcatgcttgtaatcccagctacttgagaggctgaggcaggagaatcacttgaacccgggaggcgaggttgcggtgagccgagatcgtgccattgcactctagcctgggcaaaaagagtgaaactccatctcaaataaataaataaataaataataaaaaataacttaaatctacttaattagaaaaactaacattctaaaaattttattttaagaaatatcaaaattggctgggcacggtggctcacgcctctaatccctgcactttggaaggctgaggtgggcggatcacctgaggtcaggagggtcaggagtacaagaccagcctggccaacatggcgaaaccctgtctccactaaaaatacaaaaattagccaggcatgatgatgggcacctgtaatcccagctactcaggaggctgagacagaagaatcgcttgaacccaggaggtagaggttgcagtgagctgagatcaccccactgcactccagcctgggtgacagagtgaaactccgcctcaaaaaaaaaaaaaagagaaaagaaatatagaaattaaagcatacatggccaggcgtagtggctcatgtctgtaatcccagcactttgggaggctgaggcaggcagatcacttgaggccatgagttcaagaccaacctggccaacatggcgaaagcctgtctctactaaaaatacaaaaaaattagttgggcatggtggtgcacacctgtaatcacagctactttggaggctgaggcaggagaatcgtttgaacccagaggtggaggttgcagtgagccgagattgtgccactgcactctatcctgggtgacagagcgagatactgtctcaaaaagaaaaaaaaaaggctgggcgcggtagttcatgcctgcaatcccagcactttgggaggccgaggcaggcagattacgaagtcaggagatggagaccatcctggctaatacagtgaaaccccgtctctactaaaaaatacacaaaaattagctgggtgtggtggcaggcacctgtagtcccagctactctggaggctgaggcaggagaatggcatgaacccgggaggtggagcttgcagtgagcagagatcacaccactgcactccagtctgggcgacagagcgaggctctgtctcaaaaaaaaaaaagaaagcatactctcacctccttcagtgactgatgttagtattttggcacattctttttctgtgacatatacacacttaccttgtaagtgttgtactcatttcctatgacagtaaatagtctttgtaacaggctgcatgatatttcataaaatgaatggatgtggcataatttatatgtgagccttttgaattctgctattataattaatattgcaatgaacaattcttatattgcctctacacctcaaatgtcttatcatttcttctagtttttctgaggatgtcagattattgggttaaaggatatgaacatttttaaggccttggaacagatttctaaattgctttccagaataattcccatgtgatactttcaccatgtttatttcagacttttttttttttttttttttgagacgaaatctcactctgtcacccaggctggagtgtagtggcatgatctcggctcactgcaacctccgcctcctgagtttaagcgattattctgcctcagcctcccaagtagctgcggttacaggcaagtgcctccatgcctggctaatttttgtgtcttttgtagacatggggtttcaccatgttgcccaggctggtttcgaactcctgagctcaggcaatctgcctacctcggcctcccaaagttctgggattacaggcgtgcaccaccgcgcccagccatcagagtcttttttgtcaaaataaaatggtctaaagacatacatcatagagaaactataatacaaaatttacaggtatatctaagaaaagaaaagtatatttaaagcataaaaataaactgctcttttacttaaaattttttaaaaactggattaaaaatatgaaacttccaacaaattgagcttttttttttttttttttcttttttgagacgaggtctcgcttttgtcacccagtctggagtgcagtggcgcgatctcggctcactgcaacctccacctccctggttcaagcaattcccctgcctcagcctcccaagtagctgggattacaggcgcatgccaccacgtcgggctaatttttttgtatttttagtagagagggggtttcaccatgttggccagactggtctcgaactcctgatctcaggcaatctgccagcctgggtctcccaacatgctgggattacaggcatgagccactgcactcggcctgaactttttatagtagtaacgataattcagtaatgtccaataatgactaagtaagttataacaagtacaatgtcagcaataactagtgctttttagtaaacagggtcaggcaaccttgtacccttttaaaaatgttcgaatatcgatatacctccttcctacttggtggaggattgattgaggaggaaagtgtgcagtgatggttaccagcttcagcctcttggcttgactttgcaaatactggtgagaatttggaaagagcttgagaatatcttacatagtcacatgttgctgagaagagttaagaactaacttcttgatgttcatttttaacaatggcttgcattcaaaaccttgtagagctcattagtaggagctaagaagctaatatttgcctttcactaaaattcctgattacttagcctaggtagttcgttgtctctctaggttctgtctttgggagcttgggtctaaggttatcaagctaactctttcttccctctcacccttcccaaattgaccctggtgctgatttgttattcatacgattttctagtttttcttttccctttttgagtatttgaagcttcatactgaatatagtaatcatagtattcatgcataaagaaaatcataaagtaattgcataaatgcataaagtaatcatagttttcatgcattaaaaaaactagttttggctgggcgctatggctcacgcttgtaatcccagcactttcggaggccaaggcaggcgaatcatctgaggtcaggagttcgagactagcctggccaacatggcgaaacctcttctctactaaaaatacaaaaaaattagccgagtatggtggcgggcgcctgtaatcctagctatttggcaggctgaggcaggagaatcacttgaacctgggaggcagaggttgcagtgagccgaggttgtgccattgcactacagcctaggcgacaagagcaagactccatctcaaaaaaaaaaaaaaaaaaaaaaaaactccctattacagattcataatttatgagtcattaaataatattttcaagccatgacattttttccagcagtagtctctaaatctgttttaccatcataaaaccccaagcaaaactctactacatcagctgtgtcactgtaaaacctgccttaactcacagaagcatgaaattaagcaatgtgtgtgaaactattttataaactgtaaagtattccatacatacatgttggcagttattaatgtcttctctaggtgtggctttgaaatggatgcagatgctttctgttacaaaaaacataagttgcaaatgttctataacaaggagagacacaaatatcttcatggacatggattgctatgagtgtttgattgcctaatacttgagccaccacttcagtgatatggtataatttatcaaacagtgttgagaaacagaaactactggggatgttttaaagaggaaaatacttaatatagaaattaggggtttacataatcttaagaaaggatgaaggtgcagctcttagccaggcctccacagtaccacaaaccaacttgcaggaagagctgtaaccactgccccagttgggacaatgggtaatgaggatattaaatttaagaacatactgctatagcaatgatccttggcatagaaagctgccaccacaattgcctagagatgggaacatgaagtctggcccccattgcaacagcagtgaagcagaattttgggactggcatctcccaaatggctttgcttgccaccagagaacaaccaaagtggagggagatggctaggcctcatttctgcctattttattttattttttgagacggagtcttgtctgtcgcccaggctggagtgcagtagtgtgatctcggctcactgcagcctccgcctcccagcttcaaacaattctcctgcctcagcctcctgagtagctgggattacaggcacccgccactgtgcccagccaattttcttatttttagtagaggtggggttttgccacgttggccaggctggtcttgaactcctgacctcaggtgatctgcccgcctcagcctcccaaagtgttgtgattacaggtatgagccaccatgcctggcccatttctcccttttttttttttttttttttttgaggtggagtctcactctgttgcccagactggagtgcagtggtgcaatcttggcgcattgcaacctctgcctcccagtttcaagcaattcttctgcttcagcctcctgagtagctgggactacaggtgtgtagcaccacacctggctaatttttgtttttgttttgttttttttgagacagagtctcactctgtcacccaggctggagtgtagtggcatgatctgggctcactacaacctccgcctcccgggttcaagcaattctcctgcctcagcctccagagtagctgggattacaggtgtgcgccaacacacctggctaatttttttgtatttttaatagagatggggtttcaccatgttggccaggctggtctcgaactcctgacctcgtgatccgcccgcctcggcctcccaaagtgctgggattacaggcatgagccaccgtgcccagacaaggtttgtatttttagtagagacagttttgccatgttggccaggctggtcttgaactcctcacctcaggtgatccgcctgccttggcctcccaaagtgctgggattacaggcgcaagccactgtgcctgacccgtttctgctttttaaagctcatgtgagcacttaatttgtaaccagaatcctacttgtaaaataatctaagacatgtagcttttagctttgtaacctctataatattgatggcacagtgggagtggatgctgagtaccacttgaacatgttccacctcagtgtcttcacagctggaaggtgtctacattgtttcaaggtggacaattgatttacttctcatttttcataaactaaaagtagaataaaggctattcctctaaaattgctatctcacctgtcactcccttgcattctcacataccttcttgagtggaggggcagagggcatggagtgatagcagatgtgccaggaattctccataactcagtccgtccctcttgtgctatgttgcagcatcaggatttgctaatgggaggatactgcccttacgtgcatcattagccatgcacactaaggtcttacacctacacacaggtcagtattctggctcagagaccaacagggagaaattgcagttctcattagttgaactttctttattgttcacagttttaaaacacaaaattgagaggaactctataaaaaatgtgccattctattaataattgttgctggtaatttaaaaatccttgttccttttcaaattcttatataccttttttttttaaacacttgatcttagccaaaagaccgagaagcaatcttttttttttttttttttttttttaacctatagcttctcactgagattgtcagctgtttgtaagttttggtttttggttttctgtgtttgtatttacatatatgaaatacagattgagtatcccttatccaaaatgcttaagactggaagtgttttagatttggggttttttaggatttgtgaatatttgcactatacttaccagttaagcattccaaatccaaaatttcaaatctgaagtgttccactgagcacctcttttgagtatcatgttggtgctcaaaaagtttctgattttggagcatttggatttctgattctcggatttaggatgcttgacctgtaatttcagatttacataaaagcagaaatagtacacagagctccttatatccttcacccagattccccaattattggcctttctgaaccatttgggaataatatgcagatatgattttccattatgtctcagttgttcagtgtatattttctaagtacaagaatatattcctacatatttacatgataaccgtcatgtttaaacattttaaaatggggatttgtattacattgtttctctttttgaaaaaattacagaggagcttaatgcaatcagtattacttaaaatctgataatgtgtgttaaatagtagttttcatttatttcatttatcaggtgttcagtgaatgcttactatgtaacagcacagttatcagcactggggaaatagatgagtaagataagatttgcactttcattagcttacatgccataaagagggaaataaagagaacaccagatgatgataagtttatgctgagaattaaaatgaagtgatgaaataatgggaatgtcaggtggctacttttggtgggatggtcaggaaaggcatctctggggagataaattttaagctcagacctgagtgaaaagaatgagccagccatggaaacattatgttaactcacatggtagtttgaaatgctttatctgatcaaaggtacttatttttggtgactttcaacaatattaagggtctataaaccaacactcatttgcataagaataactaccagtgaatctttttgtatgataggttttttgtttgttgtttttttgagacagagtctcgctctgtcgcccaggctggagtgcagtggcgcgatcttggctcactgcaacctctacctccccggttcaagtgattctcctgcctcagcctcccaaagtagctgggattacaggtgcctgccaccacgcctggctaatttttgtatttttagtagagatggggtttcaccgtgttgtccaggctcgtgtcaaacttctgacctcaagccatccacccgcctcggcctcccaaagtgctgggattacaggtgtgagccaccactcctggccatgataggttattttgtgatgaaaatacctacctcttaatttgtctgataaatttaaattttatgtctagatttcctaagatcagcacttccatattttaaagtaatctgtatcagactaactgctcttgcattcttttaataccagtgactactttgattcgtgaaacaatgtattttccttatgaatagtttttctcatggtgtatttattcttttaagttttgttttttaaatatacttcacttttgaatgtttcagacagcagcaaaagcagcaacagcagcagcagcagcagcagcagggggacctatcaggacagagttcacatccatgtgaaaggccagccaccagttcaggagcacttgggagtgatctaggtaaggcctgctcaccattcatcatgttcgctaccttcacactttatctgacatacgagctccatgtgatttttgctttacattattcttcattccctctttaatcatattaagaatcttaagtaaatttgtaatctactaaatttccctggattaaggagcagttaccaaaagaaaaaaaaaaaaaaaagctagatgtggtggctcacatctgtaatcccagcactttgggaaaccaaggcaggagaggattgctagaacatttaatgaatactttaacataataatttaaacttcacagtaatttgtacagtctccaaaaattccttagacatcatggatatttttctttttttgagatggagtcttgctctgtcacccaggctggagtgcagtgtcgcgatctcggctcactgcaagctctgcttcctgggttcatggcattctcctgcctcagcctcctgagtagctgggactacaggcgcccgccacatcgcctggctaattttttgtatttttagtagagacagggtttcaccatgttagccaggatggtctcaatctcctgacctcatgatccgcccgcctcggcctcccaaagtgctgggattacaggcgtgagccatcacgtccggccagaaatcatgaatattagtaggtgaaaaataaacacattttaccacctggaaaatgaaaaatacttgagtataatctaaataacaatgggaagtgcagagttactttccaggtctcggtttaaatatgtcttaaactttggccaattagtagtagaagttgagagaaaaagtaactatctgacaaagaaattataagcagaatatataaagaactcttaaaactgaataatcagaaaacaactcaataaaaaggtgaaggatttgaaaagatatttcaccaaataagacatagggatgacaaataagcacatgaaaagactctcagcatcactagtcacagggaaatgcacgataaaaccacagtgagacaccatggcacccctgtaggtatggctttaatgaagaaataaaactgacaataccaagtgttggcaaggatccaagcagctgagactcatatactgttaatgggaatgtaaaagtgtacagctttggaaaacagtttggcatttttttgataaatgtatacttagccatgtgatccagcagtcccaatcatgtatatataaccaaaagaaaagaaaacttaggttcacataaaaacttatatcaaatgcttatagctgaccaggcatggtggcccatgcctataatcccagcactttgggaggccgaggttggcagatacctgaagtcaagtgttcgagaccagcctggccaacatggcaaaaccctgtctctacttaaaatacaaaaattagccaggcgtgatggcaggcacctgtagtccagctattcaggaggctgaggcaggagaatcacgtgaacccgggaggcagaggttgcagtgagccgagatcgtgccactatactccagcctgggtgacagagcaaaactctgtctcaaaaaaaaaaaaaaaaaaaagggctggacacggtggcttacgcctgttatcccggcactttgggaggccaaggctgatggatcacctgaggtcaggagttcaagaccagcctggccaacatggtgaaaccccatctctactaaaaatacaaaaatttgctgggcatggtggtgggcacctgtaatcccaggaggctgaggcaggagaatcacttgaacccgggaggcggagattgcagtgagccaagattgtgccattgaactccagcctgggtgacaagaccaaaactccttctcaaaaaaaaaaaagattatagcatctttattcatcattgcccaaaattacaaactgcctaaatgtagaccttcatttagttaatgaatgcacaaactgtggtatatccaaacaattgaataaaaaaaggaatgaactggtacttttttctattcctcctgtttaagtacagccaaaacacctcaacatttgtataaaacatgagctgggctgggtgcggtggctcacacgtgtaatcccagcactttgggaggctgaggcgggtggatcacctaaggttgggagttcaagaccggtctgaccaacatggagaaaccctgtctcaactaaaaatacaagattagtcgggcatggtggcgcatgcctgtaatcccagcttcttgggaggctgaggcaggagaattgcttgatcccgggaagcgaaggttgcagtaagctgagattgcaccattgcactccagcctgggcaacaagagcaaaactctgtctcaaaaagaaaaaaaaaaccattcagctgaatctcaaaggcagagagaagacagactggctagggaccttggaaccagaggagcagtgtggtggggagtggactggattttctttttgcctcatttatcctggacttggtgctggagaagctatgggttcagaccaagagaaaaccccatgaaaagcctgctctctctagccaaaagaggcaacctagcaagataaaaacctttagataataagcacttgactccagtcaaacaaaacagaataaactggccccattcacccctgtcagcaaaggccaagtgggagccaagatatgtaccccaacctggaagtcataaggtacacttctcccctttcccagccaaggtggtgttagagaaggctgactggggagctgggattctcattccctccaggaggtgataacactcctttcacatggtgtcagtggtcacagggaggctgaacttccacccagtaatacataggcatctctctggctcctatatgggtgatgttggagaagaggccgagtagagaatccagactgttgctgacacccagcagtaacaaggacacctccacaatgtccgtggaggccatgtggagatcagtaacaaggcactgctctccctcccagtcagagagatgtcagtggaggactagggggctagaactcccatgtgcgttcagcagtaatccccatgaccgccactccttgacatcacaggccttgaagaaacctggactttcactcccctctggttgtagcgaggtggcactcccttttccctgttgccagtgctgtgtcagtggaggcttgctaaattggaagatgtaaataagattcacattctcataacataataccccaaattttcaggatttaattgaaaatcactaagctgggcatggtggctcacacctgtaatcccagcactttgggaggccaaggtgggccaaacacttaaggtcaggaattcaagaccagcctggccagcatggtgaaaccctgtctctactaaaaatacaaaaattagctgggcgtggtggcacatgcctgtaatcccagctactgggaaggctaaggcaggaaaatcactggaacctgggagacggaggttgcagtgatccaagatcgcactagtgtactgcagcctgggcaacagagcaagactccatctaaatttgtgtcaggattcccagaaggagatgagaaagggtggggctgaaaaaaattgaggaagaagtcatggctgaaaatttcccaaatttggcaaaagtcagaaacctacagattgaaaaagctgaatgaagctcaaatatgataaactcaaagaagttcacacagagacacatcacagtcagatttctgaacactgcagacaaaaaatgaagatctcgaaattagcaagaaatgaccttacctaagcaatttgaatgacagcagatttcccatcagagatcataaaggccagaaggaaggggtacatacaacattttttctagtgctgaaagacaaaaactctaggctgggcacggtggcacacacctgtaatcccagcacttttggaggctgaggcaggcagatcacctgaagtcaggagttcgagaccagcctggccaacatggggaaaccctgtctctactaaaaatacaaaaattagccaggtgtggtggcacgcacctataatcctagctacttgggaggctgaggcaggggaatcgcttgaacctgggaggcgacggttgcagtgagccaaggtcgcgccactgcactccagcctgggcagttgagcgagactccatctcaaaaaaaaaaaaattatccaggcttggtggtgggcgcctatagtcccagctacttgggaggctgaggcaagagaattggttgaacccaggaggtggaggttgcagtgagccaagctcatgccactgtactccagcctgggtgacagagcgagaccttgtctcaaaaaaaaaaaaaaaaaaaaaaaacaagaaaaaaactctaaacccagagttacatatccagtgaaatatccttcaggagtgaagggaaaattaacgatttgtcttcaggagacctaccctaaaagaatggctaaaggaatttctctaaacagaaaagaaatgataaaagaagtaattttggaacatcaggaaggaagaaagaacaataaaaagagtaaaatatgggtaaacacaatagactttcccctccttttgaattttctaaattgtatgatggttgaagcaagaattatagcactgatttggttttcagtatatatattggaaatatttaaggcattatgttacagatgaaggagggtcaaaggatataaagggaggtaacctttctatatttcttttgtactgatgcaggcactttggaaaataatttcactatttgtttaaaaactgaacataccctgaccatatgacatagcatctatactcctgggcatttatcccagagaaacagaaatttatttattttttttttagtattacactccgtaagtgctgtaatactagcacttagggaggctgaggcaagcagattgcttgagcccaggagttcaagaccagcctgggcaatgctgcacagtcaaaaaagaaaaacaaacatttagaaaactattttaaaagtctttaattgctgaatgcctctttggctaatatttggaagatcattattattatttttcttttttaggcagagtcttgctctgtcactgaggctggagtgcagtggcgccatctcggcttactgcaacctctgcctcccgggttcacgccattctcctgcctcagcctcccgagtagctgggactacaggcgtgtgccaccatgcccggctaattttttgtgtttttagtagagatggggtttcactatgttagtcaggatggtctccatctcctaacctcgtgatccgcccacctcggcttcccaaaatgctgggattacaggcgtgagccactgtgcccagcctggaagatcattatttagtcctacaactgacacattgttccactgacgcaattgcccaggctggtcttgaactcctgggctcaagcaatctgcctgcctcggcctccctaagtgctagtattacaggcttgagccactgtgcccagccaaaaatagaaatttatattctcacaaaaacatgtacatgaatgtttatagcagctttacttgtcataatcaaaaactggaaacaaccaaaatgtcctacagtgaaacaaactgtagtacatccatagcatgtaatactctactgtcaggattaaaaagaaacccactgttggcacaggcagcaccgtggctggatctcaggggcattatgctgagtgcaaaaaagcctcaaagggtcttacactgtatgattccacttgttcaactaaaaatgacagctgtatagagatagagaacatattagtggtttccactagttagagaaagtgggtaaaagataggtgggtgggaatataaatcgatagcagggagatctttgtggtattataacacttctatgtcttgattgtagtggtggtggttacatgaatacacgtgtgataaaatgccatgtagaactacatataacgttgtgccaatgtcaatatctaggttttagtttgatctttagttacataagatgtaactattgggtgaaattgggcaaaagagtacacgaaacctctcttaaatatctttacaacttcctttgaattgacagtttttcaaaatagaaagttgggtttttgtaaatacatgaattgttgatatacacaacaaatctcaaatgcattatgctacgtgaaagaagccatattcaaaaggctacatacctactgatgccttttatatgacgtgcaggaaaagataaaactgtaggacagagaatatactggtggctatctgggattaggaaatggggatcgaccacaaaggggcagcatgggggaattttctggggcaatggaatggttgtgtatcttgatggtgtatttgtcaaaatatatagaactataaaagtaaattttgctttatatgtattaaatcaaaaaaagaaactcgtgctcaaatagaaatacattttctgagaacttgccttttgatgactttgagaattttctggaaattttaaagaaatgtggttttgtttcccaacaggtgatgctatgagtgaagaagacatgcttcaggcagctgtgaccatgtctttagaaactgtcagaaatgatttgaaaacagaaggaaaaaaataatacctttaaaaaataatttagatattcatactttccaacattatcctgtgtgattacagcatagggtccactttggtaatgtgtcaaagagatgaggaaataagacttttagcggtttgcaaacaaaatgatgggaaagtggaacaatgcgtcggttgtaggactaaataatgatcttccaaatattagccaaagaggcattcagcaattaaagacatttaaaatagttttctaaatgtttctttttcttttttgagtgtgcaatatgtaacatgtctaaagttagggcatttttcttggatctttttgcagactagctaattagctctcgcctcaggctttttccatatagtttgttttctttttctgtcttgtaggtaagttggctcacatcatgtaatagtggctttcatttcttattaaccaaattaacctttcaggaaagtatctctactttcctgatgttgataatagtaatggttctagaaggatgaacagttctcccttcaactgtataccgtgtgctccagtgttttcttgtgttgttttctctgatcacaacttttctgctacctggttttcattattttcccacaattcttttgaaagatggtaatcttttctgaggtttagcgttttaagccctacgatgggatcattatttcatgactggtgcgttcctaaactctgaaatcagccttgcacaagtacttgagaataaatgagcattttttaaaatgtgtgagcatgtgctttcccagatgctttatgaatgtcttttcacttatatcaaaaccttacagctttgttgcaaccccttcttcctgcgccttattttttcctttcttctccaattgagaaaactaggagaagcatagtatgcaggcaagtctccttctgttagaagactaaacatacgtacccaccatgaatgtatgatacatgaaatttggccttcaattttaatagcagttttattttattttttctcctatgactggagctttgtgttctctttacagttgagtcatggaatgtaggtgtctgcttcacatcttttagtaggtatagcttgtcaaagatggtgatctggaacatgaaaataatttactaatgaaaatatgtttaaatttatactgtgatttgacacttgcatcatgtttagatagcttaagaacaatggaagtcacagtacttagtggatctataaataagaaagtccatagttttgataaatattctctttaattgagatgtacagagagtttcttgctgggtcaataggatagtatcattttggtgaaaaccatgtctctgaaattgatgttttagtttcagtgttccctatccctcattctccatctccttttgaagctcttttgaatgttgaattgttcataagctaaaatccaagaaatttcagctgacaacttcgaaaattataatatggtatattgccctcctggtgtgtggctgcacacattttatcagggaaagttttttgatctaggatttattgctaactaactgaaaagagaagaaaaaatatcttttatttatgattataaaatagctttttcttcgatataacagattttttaagtcattattttgtgccaatcagttttctgaagtttcccttacacaaaaggatagctttattttaaaatctaaagtttcttttaatagttaaaaatgtttcagaagaattataaaactttaaaactgcaagggatgttggagtttagtactactccctcaagatttaaaaagctaaatattttaagactgaacatttatgttaattattaccagtgtgtttgtcatattttccatggatatttgttcattacctttttccattgaaaagttacattaaacttttcatacacttgaattgatgagctacctaatataaaaatgagaaaaccaatatgcattttaaagttttaactttagagtttataaagttcatatataccctagttaaagcacttaagaaaatatggcatgtttgacttttagttcctagagagtttttgtttttgtttttgtttttttttgagacggagtcttgctatgtctcccaggctggagggcagtggcatgatctcggctcactacaacttccacctcccgggttcaagcaattctcctgcctcagcctccagagtagctgggattacaggcgcccaccaccacacccggcagatttttgtatttttggtagagacgcggtttcatcatgtttggccaggctggtctcgaactcctgacctcaggtgatccgcctgccttggcctcccaaagtgttgggattacaggcatgagccactgcgcctggccagctagagagtttttaaagcagagctgagcacacactggatgcgtttgaatgtgtttgtgtagtttgttgtgaaattgttacatttagcaggcagatccagaagcactagtgaactgtcatcttggtggggttggcttaaatttaattgactgtttagattccatttcttaattgattggccagtatgaaaagatgccagtgcaagtaaccatagtatcaaaaaagttaaaaattattcaaagctatagtttatacatcaggtactgccatttactgtaaaccacctgcaagaaagtcaggaacaactaaattcacaagaactgtcctgctaagaagtgtattaaagatttccattttgttttactaattgggaacatcttaatgtttaatatttaaactattggtatcatttttctaatgtataatttgtattactgggatcaagtatgtacagtggtgatgctagtagaagtttaagccttggaaataccactttcatattttcagatgtcatggatttaatgagtaatttatgtttttaaaattcagaatagttaatctctgatctaaaaccatcaatctatgttttttacggtaatcatgtaaatatttcagtaatataaactgtttgaaaaggctgctgcaggtaaactctatactaggatcttggccaaataatttacaattcacagaatattttatttaaggtggtgctttttttttttgtccttaaaacttgatttttcttaactttattcatgatgccaaagtaaatgaggaaaaaaactcaaaaccagttgagtatcattgcagacaaaactaccagtagtccatattgtttaatattaagttgaataaaataaattttatttcagtcagagcctaaatcacattttgattgtctgaatttttgatactatttttaaaatcatgctagtggcggctgggcgtggtagctcacgcctgtaatcccagcattttgggaggccgaagtgggtggatcacgaggtcgggagttcgagaccagcttggccaaaatggtgaaaccccatctgtactaaaaactacaaaaattagctgggcgcggtggcaggtgcctgtaatcccagctacctgggagtctgaggcaggagaattgcttgaaccctggcgacagaggatgcagtgagccaagatggtgccactgtactccagactgggcgacagagtgagactctgtctcaaaaaaaaaaaaaaaatcatgctagtgccaagagctactaaattcttaaaaccggcccattggacctgtacagataaaaaatagattcagtgcataatcaaaatatgataattttaaaatcttaagtagaaaaataaatcttgatgttttaaattcttacgaggattcaatagttaatattgatgatctcccggctgggtgcagtggctcacgcctgtaatcccagcagttctggaggctgaggtgggcgaatcacttcaggccaggagttcaagaccagtctgggcaacatggtgaaacctcgtttctactaaaaatacaaaaattagccgggcgtggttgcacacacttgtaatcccagctactcaggaggctaagaatcgcatgagcctaggaggcagaggttgcagagtgccaagggctcaccactgcattccagcctgcccaacagagtgagacactgtttctgaaaaaaaaaaatatatatatatatatatatatgtgtgtatatatatatgtatatatatatgacttcctattaaaaactttatcccagtcgggggcagtggctcacgcctgtaatcccaacactttgggaggctgaggcaggtggatcacctgaagtccggagtttgagaccagcctggccaacatggtgaaaccccatctctactaaaaatacaaaacttaagccaggtatggtggcgggcacctgtaatcccagttacttgggaggctgaggcaggagaatcgtttaaacccaggaggtggaggttgcagtgagctgagatcgtgccattgcactctagcctgggcaacaagagtaaaactccatcttaaaggtttgtttgtttttttttaatccggaaacgaagaggcgttgggccgctattttctttttctttctttctttctttctttttttttttttctgagacggagtctagctctgctgcccaggctggagtacaatgacacgatgttggctcactgcaacctccacctcctgggttcaagcgattctcctgcctcagcctcccaagtacctgggattacaggcacctgccactacacctggcgaatatttgttttttttagtagagacgggcttttaccatgttaggctggtctcaaactcctgacctcaggtgatctgcctgccttggcctcccaaagtgctgggattacaggtgcaggccaccacacccggccttgggccactgttttcaaagtgaattgtttgttgtatcgagtccttaagtatggatatatatgtgaccctaattaagaactaccagattggatcaactaatcatgtcagcaatgtaaataactttatttttcatattcaaaataaaaactttcttttatttctggcccctttataaccagcatctttttgctttaaaaaatgacctggctttgtatttttttagtcttaaacataataaaaatatttttgttctaatttgctttcatgagtgaagattattgacatcgttggtaaattctagaattttgattttgttttttaatttgaagaaaatctttgctattattattttttccaagtggtctggcattttaagaattagtgctaataacgtaacttctaaatttgtcgtaattggcatgtttaatagcatatcaaaaaacattttaagcctgtggattcatagacaaagcaatgagaaacattagtaaaatataaatggatattcctgatgcatttaggaagctctcaattgtctcttgcatagttcaaggaatgttttctgaatttttttaatgctttttttttttttgaaagaggaaaacatacatttttaaatgtgattatctaatttttacaacactgggctattaggaataactttttaaaaattactgttctgtataaatatttgaaattcaagtacagaaaatatctgaaacaaaaagcattgttgtttggccatgatacaagtgcactgtggcagtgccgcttgctcaggacccagccctgcagcccttctgtgtgtgctccctcgttaagttcatttgctgttattacacacacaggccttcctgtctggtcgttagaaaagccgggcttccaaagcactgttgaacacaggattctgttgttagtgtggatgttcaatgagttgtattttaaatatcaaagattattaaataaagataatgtttgcttttcta

SEQ ID NO: 2 - DNA, 6884 bp, Homo sapiens
gtgggggccgttggctccagacaaataaacatggagtccatcttccacgagaaacaagaaggctcactttgtgctcaacattgcctgaataacttattgcaaggagaatattttagccctgtggaattatcctcaattgcacatcagctggatgaggaggagaggatgagaatggcagaaggaggagttactagtgaagattatcgcacgtttttacagcagccttctggaaatatggatgacagtggttttttctctattcaggttataagcaatgccttgaaagtttggggtttagaactaatcctgttcaacagtccagagtatcagaggctcaggatcgatcctataaatgaaagatcatttatatgcaattataaggaacactggtttacagttagaaaattaggaaaacagtggtttaacttgaattctctcttgacgggtccagaattaatatcagatacatatcttgcacttttcttggctcaattacaacaggaaggttattctatatttgtcgttaagggtgatctgccagattgcgaagctgaccaactcctgcagatgattagggtccaacagatgcatcgaccaaaacttattggagaagaattagcacaactaaaagagcaaagagtccataaaacagacctggaacgagtgttagaagcaaatgatggctcaggaatgttagacgaagatgaggaggatttgcagagggctctggcactaagtcgccaagaaattgacatggaagatgaggaagcagatctccgcagggctattcagctaagtatgcaaggtagttccagaaacatatctcaagatatgacacagacatcaggtacaaatcttacttcagaagagcttcggaagagacgagaagcctactttgaaaaacagcagcaaaagcagcaacagcagcagcagcagcagcagcagggggacctatcaggacagagttcacatccatgtgaaaggccagccaccagttcaggagcacttgggagtgatctaggtgatgctatgagtgaagaagacatgcttcaggcagctgtgaccatgtctttagaaactgtcagaaatgatttgaaaacagaaggaaaaaaataatacctttaaaaaataatttagatattcatactttccaacattatcctgtgtgattacagcatagggtccactttggtaatgtgtcaaagagatgaggaaataagacttttagcggtttgcaaacaaaatgatgggaaagtggaacaatgcgtcggttgtaggactaaataatgatcttccaaatattagccaaagaggcattcagcaattaaagacatttaaaatagttttctaaatgtttctttttcttttttgagtgtgcaatatgtaacatgtctaaagttagggcatttttcttggatctttttgcagactagctaattagctctcgcctcaggctttttccatatagtttgttttctttttctgtcttgtaggtaagttggctcacatcatgtaatagtggctttcatttcttattaaccaaattaacctttcaggaaagtatctctactttcctgatgttgataatagtaatggttctagaaggatgaacagttctcccttcaactgtataccgtgtgctccagtgttttcttgtgttgttttctctgatcacaacttttctgctacctggttttcattattttcccacaattcttttgaaagatggtaatcttttctgaggtttagcgttttaagccctacgatgggatcattatttcatgactggtgcgttcctaaactctgaaatcagccttgcacaagtacttgagaataaatgagcattttttaaaatgtgtgagcatgtgctttcccagatgctttatgaatgtcttttcacttatatcaaaaccttacagctttgttgcaaccccttcttcctgcgccttattttttcctttcttctccaattgagaaaactaggagaagcatagtatgcaggcaagtctccttctgttagaagactaaacatacgtacccaccatgaatgtatgatacatgaaatttggccttcaattttaatagcagttttattttattttttctcctatgactggagctttgtgttctctttacagttgagtcatggaatgtaggtgtctgcttcacatcttttagtaggtatagcttgtcaaagatggtgatctggaacatgaaaataatttactaatgaaaatatgtttaaatttatactgtgatttgacacttgcatcatgtttagatagcttaagaacaatggaagtcacagtacttagtggatctataaataagaaagtccatagttttgataaatattctctttaattgagatgtacagagagtttcttgctgggtcaataggatagtatcattttggtgaaaaccatgtctctgaaattgatgttttagtttcagtgttccctatccctcattctccatctccttttgaagctcttttgaatgttgaattgttcataagctaaaatccaagaaatttcagctgacaacttcgaaaattataatatggtatattgccctcctggtgtgtggctgcacacattttatcagggaaagttttttgatctaggatttattgctaactaactgaaaagagaagaaaaaatatcttttatttatgattataaaatagctttttcttcgatataacagattttttaagtcattattttgtgccaatcagttttctgaagtttcccttacacaaaaggatagctttattttaaaatctaaagtttcttttaatagttaaaaatgtttcagaagaattataaaactttaaaactgcaagggatgttggagtttagtactactccctcaagatttaaaaagctaaatattttaagactgaacatttatgttaattattaccagtgtgtttgtcatattttccatggatatttgttcattacctttttccattgaaaagttacattaaacttttcatacacttgaattgatgagctacctaatataaaaatgagaaaaccaatatgcattttaaagttttaactttagagtttataaagttcatatataccctagttaaagcacttaagaaaatatggcatgtttgacttttagttcctagagagtttttgtttttgtttttgtttttttttgagacggagtcttgctatgtctcccaggctggagggcagtggcatgatctcggctcactacaacttccacctcccgggttcaagcaattctcctgcctcagcctccagagtagctgggattacaggcgcccaccaccacacccggcagatttttgtatttttggtagagacgcggtttcatcatgtttggccaggctggtctcgaactcctgacctcaggtgatccgcctgccttggcctcccaaagtgttgggattacaggcatgagccactgcgcctggccagctagagagtttttaaagcagagctgagcacacactggatgcgtttgaatgtgtttgtgtagtttgttgtgaaattgttacatttagcaggcagatccagaagcactagtgaactgtcatcttggtggggttggcttaaatttaattgactgtttagattccatttcttaattgattggccagtatgaaaagatgccagtgcaagtaaccatagtatcaaaaaagttaaaaattattcaaagctatagtttatacatcaggtactgccatttactgtaaaccacctgcaagaaagtcaggaacaactaaattcacaagaactgtcctgctaagaagtgtattaaagatttccattttgttttactaattgggaacatcttaatgtttaatatttaaactattggtatcatttttctaatgtataatttgtattactgggatcaagtatgtacagtggtgatgctagtagaagtttaagccttggaaataccactttcatattttcagatgtcatggatttaatgagtaatttatgtttttaaaattcagaatagttaatctctgatctaaaaccatcaatctatgttttttacggtaatcatgtaaatatttcagtaatataaactgtttgaaaaggctgctgcaggtaaactctatactaggatcttggccaaataatttacaattcacagaatattttatttaaggtggtgctttttttttttgtccttaaaacttgatttttcttaactttattcatgatgccaaagtaaatgaggaaaaaaactcaaaaccagttgagtatcattgcagacaaaactaccagtagtccatattgtttaatattaagttgaataaaataaattttatttcagtcagagcctaaatcacattttgattgtctgaatttttgatactatttttaaaatcatgctagtggcggctgggcgtggtagctcacgcctgtaatcccagcattttgggaggccgaagtgggtggatcacgaggtcgggagttcgagaccagcttggccaaaatggtgaaaccccatctgtactaaaaactacaaaaattagctgggcgcggtggcaggtgcctgtaatcccagctacctgggagtctgaggcaggagaattgcttgaaccctggcgacagaggatgcagtgagccaagatggtgccactgtactccagactgggcgacagagtgagactctgtctcaaaaaaaaaaaaaaaatcatgctagtgccaagagctactaaattcttaaaaccggcccattggacctgtacagataaaaaatagattcagtgcataatcaaaatatgataattttaaaatcttaagtagaaaaataaatcttgatgttttaaattcttacgaggattcaatagttaatattgatgatctcccggctgggtgcagtggctcacgcctgtaatcccagcagttctggaggctgaggtgggcgaatcacttcaggccaggagttcaagaccagtctgggcaacatggtgaaacctcgtttctactaaaaatacaaaaattagccgggcgtggttgcacacacttgtaatcccagctactcaggaggctaagaatcgcatgagcctaggaggcagaggttgcagagtgccaagggctcaccactgcattccagcctgcccaacagagtgagacactgtttctgaaaaaaaaaaatatatatatatatatatatatgtgtgtatatatatatgtatatatatatgacttcctattaaaaactttatcccagtcgggggcagtggctcacgcctgtaatcccaacactttgggaggctgaggcaggtggatcacctgaagtccggagtttgagaccagcctggccaacatggtgaaaccccatctctactaaaaatacaaaacttaagccaggtatggtggcgggcacctgtaatcccagttacttgggaggctgaggcaggagaatcgtttaaacccaggaggtggaggttgcagtgagctgagatcgtgccattgcactctagcctgggcaacaagagtaaaactccatcttaaaggtttgtttgtttttttttaatccggaaacgaagaggcgttgggccgctattttctttttctttctttctttctttctttttttttttttctgagacggagtctagctctgctgcccaggctggagtacaatgacacgatgttggctcactgcaacctccacctcctgggttcaagcgattctcctgcctcagcctcccaagtacctgggattacaggcacctgccactacacctggcgaatatttgttttttttagtagagacgggcttttaccatgttaggctggtctcaaactcctgacctcaggtgatctgcctgccttggcctcccaaagtgctgggattacaggtgcaggccaccacacccggccttgggccactgttttcaaagtgaattgtttgttgtatcgagtccttaagtatggatatatatgtgaccctaattaagaactaccagattggatcaactaatcatgtcagcaatgtaaataactttatttttcatattcaaaataaaaactttcttttatttctggcccctttataaccagcatctttttgctttaaaaaatgacctggctttgtatttttttagtcttaaacataataaaaatatttttgttctaatttgctttcatgagtgaagattattgacatcgttggtaaattctagaattttgattttgttttttaatttgaagaaaatctttgctattattattttttccaagtggtctggcattttaagaattagtgctaataacgtaacttctaaatttgtcgtaattggcatgtttaatagcatatcaaaaaacattttaagcctgtggattcatagacaaagcaatgagaaacattagtaaaatataaatggatattcctgatgcatttaggaagctctcaattgtctcttgcatagttcaaggaatgttttctgaatttttttaatgctttttttttttttgaaagaggaaaacatacatttttaaatgtgattatctaatttttacaacactgggctattaggaataactttttaaaaattactgttctgtataaatatttgaaattcaagtacagaaaatatctgaaacaaaaagcattgttgtttggccatgatacaagtgcactgtggcagtgccgcttgctcaggacccagccctgcagcccttctgtgtgtgctccctcgttaagttcatttgctgttattacacacacaggccttcctgtctggtcgttagaaaagccgggcttccaaagcactgttgaacacaggattctgttgttagtgtggatgttcaatgagttgtattttaaatatcaaagattattaaataaagataatgtttgcttttcta

SEQ ID NO: 3 - DNA, 18 bp, Artificial sequence
  Synthetic oligonucleotide
  modified_base (2),(13),(15)..(18): m5c
gcgtaggtgatgctcccc

SEQ ID NO: 4 - DNA, 18 bp, Artificial sequence
  Synthetic oligonucleotide
  modified_base (7),(8),(10),(11),(18): m5c
aggaatcctccgaaaagc

SEQ ID NO: 5 - DNA, 18 bp, Artificial sequence
  Synthetic oligonucleotide
  modified_base (8),(9),(11),(12): m5c
aaggaatcctccgaaaag

SEQ ID NO: 6 - DNA, 18 bp, Artificial sequence
  Synthetic oligonucleotide
  modified_base (10),(11),(13),(14): m5c
tgaaggaatcctccgaaa

SEQ ID NO: 7 - DNA, 18 bp, Artificial sequence
  Synthetic oligonucleotide
  modified_base (11),(12),(14),(15): m5c
gtgaaggaatcctccgaa

SEQ ID NO: 8 - DNA, 18 bp, Artificial sequence
  Synthetic oligonucleotide
  modified_base (12),(13),(15),(16): m5c
ggtgaaggaatcctccga

SEQ ID NO: 9 - DNA, 18 bp, Artificial sequence
  Synthetic oligonucleotide
  modified_base (13),(14),(16),(17): m5c
gggtgaaggaatcctccg

SEQ ID NO: 10 - DNA, 18 bp, Artificial sequence
  Synthetic oligonucleotide
  modified_base (3),(5),(6): m5c
gactccaatatagaattg

SEQ ID NO: 11 - DNA, 18 bp, Artificial sequence
  Synthetic oligonucleotide
  modified_base (3),(7),(8),(9),(12): m5c
gtcaggccctacagtggg

SEQ ID NO: 12 - DNA, 18 bp, Artificial sequence
  Synthetic oligonucleotide
  modified_base (4),(8),(9),(10),(13): m5c
tgtcaggccctacagtgg

SEQ ID NO: 13 - DNA, 18 bp, Artificial sequence
  Synthetic oligonucleotide
  modified_base (1),(4),(7),(8),(9): m5c
cgacttccctgtttaggg

SEQ ID NO: 14 - DNA, 18 bp, Artificial sequence
  Synthetic oligonucleotide
  modified_base (2),(5),(8),(9),(10): m5c
acgacttccctgtttagg

SEQ ID NO: 15 - DNA, 18 bp, Artificial sequence
  Synthetic oligonucleotide
  modified_base (3),(6),(9),(10),(11): m5c
gacgacttccctgtttag

SEQ ID NO: 16 - DNA, 18 bp, Artificial sequence
  Synthetic oligonucleotide
  modified_base (2),(3),(6),(8),(9): m5c
gcctgctccggaaagatg

SEQ ID NO: 17 - DNA, 18 bp, Artificial sequence
  Synthetic oligonucleotide
  modified_base (13): m5c
agtagtgtggaacatgtt

SEQ ID NO: 18 - DNA, 18 bp, Artificial sequence
  Synthetic oligonucleotide
  modified_base (15): m5c
gaagtagtgtggaacatg

SEQ ID NO: 19 - DNA, 18 bp, Artificial sequence
  Synthetic oligonucleotide
  modified_base (16): m5c
ggaagtagtgtggaacat

SEQ ID NO: 20 - DNA, 18 bp, Artificial sequence
  Synthetic oligonucleotide
  modified_base (17): m5c
aggaagtagtgtggaaca

SEQ ID NO: 21 - DNA, 18 bp, Artificial sequence
  Synthetic oligonucleotide
  modified_base (1),(18): m5c
caggaagtagtgtggaac

SEQ ID NO: 22 - DNA, 18 bp, Artificial sequence
  Synthetic oligonucleotide
  modified_base (3),(4),(5),(8),(16): m5c
gtcccaactaggtaacaa

SEQ ID NO: 23 - DNA, 18 bp, Artificial sequence
  Synthetic oligonucleotide
  modified_base (2),(18): m5c
tcgggtaagtagattttc

SEQ ID NO: 24 - DNA, 18 bp, Artificial sequence
  Synthetic oligonucleotide
  modified_base (3),(4),(10),(12),(16): m5c
aggcctatacacatgctg

SEQ ID NO: 25 - DNA, 18 bp, Artificial sequence
  Synthetic oligonucleotide
  modified_base (8),(15),(16): m5c
gaagtatctgtaggccta

SEQ ID NO: 26 - DNA, 18 bp, Artificial sequence
  Synthetic oligonucleotide
  modified_base (4): m5c
ggactgtataggagatta

SEQ ID NO: 27 - DNA, 18 bp, Artificial sequence
  Synthetic oligonucleotide
  modified_base (8): m5c
gaatggactgtataggag

SEQ ID NO: 28 - DNA, 18 bp, Artificial sequence
  Synthetic oligonucleotide
  modified_base (1),(2),(4),(11),(13),(15),(16): m5c
cctcttagtgctctccga

SEQ ID NO: 29 - DNA, 18 bp, Artificial sequence
  Synthetic oligonucleotide
  modified_base (2),(3),(5),(12),(14),(16),(17): m5c
tcctcttagtgctctccg

SEQ ID NO: 30 - DNA, 18 bp, Artificial sequence
  Synthetic oligonucleotide
  modified_base (4),(8),(12),(16): m5c
aagctgtcaatctagcag

SEQ ID NO: 31 - DNA, 18 bp, Artificial sequence
  Synthetic oligonucleotide
  modified_base (5),(9),(13),(17): m5c
gggacaagctgtcaatct

SEQ ID NO: 32 - DNA, 18 bp, Artificial sequence
  Synthetic oligonucleotide
  modified_base (5),(6),(7),(11),(14): m5c
taggcccagacttcattg

SEQ ID NO: 33 - DNA, 18 bp, Artificial sequence
  Synthetic oligonucleotide
  modified_base (6),(7),(8),(12),(15): m5c
ttaggcccagacttcatt

SEQ ID NO: 34 - DNA, 18 bp, Artificial sequence
  Synthetic oligonucleotide
  modified_base (7),(8),(9),(13),(16): m5c
tttaggcccagacttcat

SEQ ID NO: 35 - DNA, 18 bp, Artificial sequence
  Synthetic oligonucleotide
  modified_base (1),(7),(14),(15),(16),(18): m5c
caatgacaatgagcccac

SEQ ID NO: 36 - DNA, 18 bp, Artificial sequence
  Synthetic oligonucleotide
  modified_base (12): m5c
gttataggatgcaggtaa

SEQ ID NO: 37 - DNA, 18 bp, Artificial sequence
  Synthetic oligonucleotide
  modified_base (13): m5c
ggttataggatgcaggta

SEQ ID NO: 38 - DNA, 18 bp, Artificial sequence
  Synthetic oligonucleotide
  modified_base (14): m5c
aggttataggatgcaggt

SEQ ID NO: 39 - DNA, 18 bp, Artificial sequence
  Synthetic oligonucleotide
ataatgggaggttatagg

SEQ ID NO: 40 - DNA, 18 bp, Artificial sequence
  Synthetic oligonucleotide
  modified_base (11),(18): m5c
gaataagtagcttggagc

SEQ ID NO: 41 - DNA, 18 bp, Artificial sequence
  Synthetic oligonucleotide
  modified_base (16): m5c
gtaaggaataagtagctt

SEQ ID NO: 42 - DNA, 18 bp, Artificial sequence
  Synthetic oligonucleotide
  modified_base (3),(5),(6),(14),(15),(16),(17): m5c
gacaccaggtttgcccct

SEQ ID NO: 43 - DNA, 18 bp, Artificial sequence
  Synthetic oligonucleotide
  modified_base (4),(6),(7),(15),(16),(17),(18): m5c
agacaccaggtttgcccc

SEQ ID NO: 44 - DNA, 18 bp, Artificial sequence
  Synthetic oligonucleotide
  modified_base (15),(18): m5c
atgggaggtaggtacaac

SEQ ID NO: 45 - DNA, 18 bp, Artificial sequence
  Synthetic oligonucleotide
  modified_base (4),(7),(9),(10),(11),(15),(17): m5c
ggactgcacccaagctca

SEQ ID NO: 46 - DNA, 18 bp, Artificial sequence
  Synthetic oligonucleotide
  modified_base (8),(11),(13),(14),(15): m5c
agagggactgcacccaag

SEQ ID NO: 47 - DNA, 18 bp, Artificial sequence
  Synthetic oligonucleotide
  modified_base (9),(12),(14),(15),(16): m5c
aagagggactgcacccaa

SEQ ID NO: 48 - DNA, 18 bp, Artificial sequence
  Synthetic oligonucleotide
  modified_base (1),(2),(3),(4),(6),(8): m5c
ccccactctaatatgaag

SEQ ID NO: 49 - DNA, 18 bp, Artificial sequence
  Synthetic oligonucleotide
  modified_base (3),(5),(7),(18): m5c
gtcgctcaggagaggttc

SEQ ID NO: 50 - DNA, 18 bp, Artificial sequence
  Synthetic oligonucleotide
  modified_base (4),(6),(8): m5c
ggtcgctcaggagaggtt

SEQ ID NO: 51 - DNA, 18 bp, Artificial sequence
  Synthetic oligonucleotide
  modified_base (5),(7),(9): m5c
aggtcgctcaggagaggt

SEQ ID NO: 52 - DNA, 18 bp, Artificial sequence
  Synthetic oligonucleotide
  modified_base (6),(6),(10): m5c
taggtcgctcaggagagg

SEQ ID NO: 53 - DNA, 18 bp, Artificial sequence
  Synthetic oligonucleotide
  modified_base (7),(9),(11): m5c
ataggtcgctcaggagag

SEQ ID NO: 54 - DNA, 18 bp, Artificial sequence
  Synthetic oligonucleotide
  modified_base (1),(12),(14),(16): m5c
cagagataggtcgctcag

SEQ ID NO: 55 - DNA, 18 bp, Artificial sequence
  Synthetic oligonucleotide
  modified_base (2),(5),(16),(18): m5c
tctgcagagataggtcgc

SEQ ID NO: 56 - DNA, 18 bp, Artificial sequence
  Synthetic oligonucleotide
  modified_base (1),(9),(11): m5c
cggtaaagcactagatgg

SEQ ID NO: 57 - DNA, 18 bp, Artificial sequence
  Synthetic oligonucleotide
  modified_base (2),(10),(12): m5c
acggtaaagcactagatg

SEQ ID NO: 58 - DNA, 18 bp, Artificial sequence
  Synthetic oligonucleotide
  modified_base (6),(8),(16),(18): m5c
agtggcacggtaaagcac

SEQ ID NO: 59 - DNA, 18 bp, Artificial sequence
  Synthetic oligonucleotide
  modified_base (5),(10),(11),(14),(16): m5c
agtgctgggcctactctg

SEQ ID NO: 60 - DNA, 18 bp, Artificial sequence
  Synthetic oligonucleotide
  modified_base (6),(11),(12),(15),(17): m5c
aagtgctgggcctactct

SEQ ID NO: 61 - DNA, 18 bp, Artificial sequence
  Synthetic oligonucleotide
  modified_base (2),(18): m5c
gctatgttagttgtgtac

SEQ ID NO: 62 - DNA, 18 bp, Artificial sequence
  Synthetic oligonucleotide
  modified_base (3),(6),(8),(11),(14),(17): m5c
aacgtctctgcagcagct

SEQ ID NO: 63 - DNA, 18 bp, Artificial sequence
  Synthetic oligonucleotide
  modified_base (5),(17): m5c
gaagctaagtaggtgact

SEQ ID NO: 64 - DNA, 18 bp, Artificial sequence
  Synthetic oligonucleotide
  modified_base (6),(18): m5c
tgaagctaagtaggtgac

SEQ ID NO: 65 - DNA, 18 bp, Artificial sequence
  Synthetic oligonucleotide
  modified_base (11),(12),(13),(15),(17): m5c
agaggtgattcccactcg

SEQ ID NO: 66 - DNA, 18 bp, Artificial sequence
  Synthetic oligonucleotide
  modified_base (12),(13),(14),(16),(18): m5c
tagaggtgattcccactc

SEQ ID NO: 67 - DNA, 18 bp, Artificial sequence
  Synthetic oligonucleotide
  modified_base (1),(13),(14),(15),(17): m5c
ctagaggtgattcccact

SEQ ID NO: 68 - DNA, 18 bp, Artificial sequence
  Synthetic oligonucleotide
  modified_base (1),(2),(14),(15),(16),(18): m5c
cctagaggtgattcccac

SEQ ID NO: 69 - DNA, 18 bp, Artificial sequence
  Synthetic oligonucleotide
  modified_base (9),(14): m5c
ggtaatagctaagcaaga

SEQ ID NO: 70 - DNA, 18 bp, Artificial sequence
  Synthetic oligonucleotide
  modified_base (2),(7),(13): m5c
gctactctggtacaggaa

SEQ ID NO: 71 - DNA, 18 bp, Artificial sequence
  Synthetic oligonucleotide
  modified_base (1),(2),(7),(9): m5c
cctagtcactttgataga

SEQ ID NO: 72 - DNA, 18 bp, Artificial sequence
  Synthetic oligonucleotide
  modified_base (2),(4),(11),(13),(16): m5c
gcactaaaggctcatctg

SEQ ID NO: 73 - DNA, 18 bp, Artificial sequence
  Synthetic oligonucleotide
  modified_base (4),(7): m5c
gaacatcttgagtaggtg

SEQ ID NO: 74 - DNA, 18 bp, Artificial sequence
  Synthetic oligonucleotide
  modified_base (5),(8): m5c
ggaacatcttgagtaggt

SEQ ID NO: 75 - DNA, 18 bp, Artificial sequence
  Synthetic oligonucleotide
  modified_base (6),(9): m5c
aggaacatcttgagtagg

SEQ ID NO: 76 - DNA, 18 bp, Artificial sequence
  Synthetic oligonucleotide
  modified_base (1),(7),(10): m5c
caggaacatcttgagtag

SEQ ID NO: 77 - DNA, 18 bp, Artificial sequence
  Synthetic oligonucleotide
  modified_base (5): m5c
tgttcagggtagatgtca

SEQ ID NO: 78 - DNA, 18 bp, Artificial sequence
  Synthetic oligonucleotide
  modified_base (7): m5c
ggtgttcagggtagatgt

SEQ ID NO: 79 - DNA, 18 bp, Artificial sequence
  Synthetic oligonucleotide
  modified_base (8): m5c
aggtgttcagggtagatg

SEQ ID NO: 80 - DNA, 18 bp, Artificial sequence
  Synthetic oligonucleotide
  modified_base (9),(14),(18): m5c
gggtgggacataacaggc

SEQ ID NO: 81 - DNA, 18 bp, Artificial sequence
  Synthetic oligonucleotide
  modified_base (10),(15): m5c
agggtgggacataacagg

SEQ ID NO: 82 - DNA, 18 bp, Artificial sequence
  Synthetic oligonucleotide
  modified_base (6),(8),(11),(12),(13),(18): m5c
ggatactctgccctgttc

SEQ ID NO: 83 - DNA, 18 bp, Artificial sequence
  Synthetic oligonucleotide
  modified_base (7),(9),(12),(13),(14): m5c
tggatactctgccctgtt

SEQ ID NO: 84 - DNA, 18 bp, Artificial sequence
  Synthetic oligonucleotide
  modified_base (4),(11),(14),(16),(18): m5c
aagctagatgctacacac

SEQ ID NO: 85 - DNA, 18 bp, Artificial sequence
  Synthetic oligonucleotide
  modified_base (1),(5),(16): m5c
caaacgtgtggtttgcat

SEQ ID NO: 86 - DNA, 18 bp, Artificial sequence
  Synthetic oligonucleotide
  modified_base (2),(6),(17): m5c
tcaaacgtgtggtttgca

SEQ ID NO: 87 - DNA, 18 bp, Artificial sequence
  Synthetic oligonucleotide
  modified_base (3),(7),(18): m5c
gtcaaacgtgtggtttgc

SEQ ID NO: 88 - DNA, 18 bp, Artificial sequence
  Synthetic oligonucleotide
  modified_base (4),(8): m5c
tgtcaaacgtgtggtttg

SEQ ID NO: 89 - DNA, 18 bp, Artificial sequence
  Synthetic oligonucleotide
  modified_base (6),(10): m5c
ggtgtcaaacgtgtggtt

SEQ ID NO: 90 - DNA, 18 bp, Artificial sequence
  Synthetic oligonucleotide
  modified_base (4),(5),(8),(9): m5c
gtaccttcctgtgatggt

SEQ ID NO: 91 - DNA, 18 bp, Artificial sequence
  Synthetic oligonucleotide
  modified_base (1),(5),(8),(10),(12),(16): m5c
caggctactcacttactg

SEQ ID NO: 92 - DNA, 18 bp, Artificial sequence
  Synthetic oligonucleotide
  modified_base (2),(6),(9),(11),(13),(17): m5c
gcaggctactcacttact

SEQ ID NO: 93 - DNA, 18 bp, Artificial sequence
  Synthetic oligonucleotide
  modified_base (3),(7),(10),(12),(14),(18): m5c
agcaggctactcacttac

SEQ ID NO: 94 - DNA, 18 bp, Artificial sequence
  Synthetic oligonucleotide
  modified_base (4),(8),(11),(13),(15): m5c
gagcaggctactcactta

SEQ ID NO: 95 - DNA, 18 bp, Artificial sequence
  Synthetic oligonucleotide
  modified_base (5),(9),(12),(14),(16): m5c
tgagcaggctactcactt

SEQ ID NO: 96 - DNA, 18 bp, Artificial sequence
  Synthetic oligonucleotide
  modified_base (4),(10),(14),(17): m5c
ttgactgagcaggctact

SEQ ID NO: 97 - DNA, 18 bp, Artificial sequence
  Synthetic oligonucleotide
  modified_base (1),(6),(11),(15),(18): m5c
cttgactgagcaggctac

SEQ ID NO: 98 - DNA, 18 bp, Artificial sequence
  Synthetic oligonucleotide
  modified_base (2),(7),(12),(16): m5c
acttgactgagcaggcta

SEQ ID NO: 99 - DNA, 18 bp, Artificial sequence
  Synthetic oligonucleotide
  modified_base (1),(5),(6),(7),(10),(11): m5c
caggcccttccatagtgt

SEQ ID NO: 100 - DNA, 18 bp, Artificial sequence
  Synthetic oligonucleotide
  modified_base (1),(2),(6),(7),(8),(11),(12): m5c
ccaggcccttccatagtg

SEQ ID NO: 101 - DNA, 18 bp, Artificial sequence
  Synthetic oligonucleotide
  modified_base (2),(3),(7),(8),(9),(12),(13): m5c
tccaggcccttccatagt

SEQ ID NO: 102 - DNA, 18 bp, Artificial sequence
  Synthetic oligonucleotide
  modified_base (1),(7): m5c
cgtgtgctagtatttgtt

SEQ ID NO: 103 - DNA, 18 bp, Artificial sequence
  Synthetic oligonucleotide
  modified_base (1),(2),(8): m5c
ccgtgtgctagtatttgt

SEQ ID NO: 104 - DNA, 18 bp, Artificial sequence
  Synthetic oligonucleotide
  modified_base (3),(4),(10): m5c
ggccgtgtgctagtattt

SEQ ID NO: 105 - DNA, 18 bp, Artificial sequence
  Synthetic oligonucleotide
  modified_base (4),(5),(11): m5c
tggccgtgtgctagtatt

SEQ ID NO: 106 - DNA, 18 bp, Artificial sequence
  Synthetic oligonucleotide
  modified_base (5),(6),(12): m5c
ttggccgtgtgctagtat

SEQ ID NO: 107 - DNA, 18 bp, Artificial sequence
  Synthetic oligonucleotide
  modified_base (6),(7),(13): m5c
attggccgtgtgctagta

SEQ ID NO: 108 - DNA, 18 bp, Artificial sequence
  Synthetic oligonucleotide
  modified_base (7),(8),(14): m5c
gattggccgtgtgctagt

SEQ ID NO: 109 - DNA, 18 bp, Artificial sequence
  Synthetic oligonucleotide
  modified_base (8),(9),(13),(14),(15): m5c
aaggttgcctgaccctgt

SEQ ID NO: 110 - DNA, 18 bp, Artificial sequence
  Synthetic oligonucleotide
  modified_base (1),(9),(10),(14),(15),(16): m5c
caaggttgcctgaccctg

SEQ ID NO: 111 - DNA, 18 bp, Artificial sequence
  Synthetic oligonucleotide
  modified_base (2),(10),(11),(15),(16),(17): m5c
acaaggttgcctgaccct

SEQ ID NO: 112 - DNA, 18 bp, Artificial sequence
  Synthetic oligonucleotide
  modified_base (5),(13),(14),(18): m5c
ggtacaaggttgcctgac

SEQ ID NO: 113 - DNA, 18 bp, Artificial sequence
  Synthetic oligonucleotide
  modified_base (6),(14),(15): m5c
gggtacaaggttgcctga

SEQ ID NO: 114 - DNA, 18 bp, Artificial sequence
  Synthetic oligonucleotide
  modified_base (14): m5c
tagtagagttttgcttgg

SEQ ID NO: 115 - DNA, 18 bp, Artificial sequence
  Synthetic oligonucleotide
  modified_base (18): m5c
gatgtagtagagttttgc

SEQ ID NO: 116 - DNA, 18 bp, Artificial sequence
  Synthetic oligonucleotide
tgatgtagtagagttttg

SEQ ID NO: 117 - DNA, 18 bp, Artificial sequence
  Synthetic oligonucleotide
  modified_base (1): m5c
ctgatgtagtagagtttt

SEQ ID NO: 118 - DNA, 18 bp, Artificial sequence
  Synthetic oligonucleotide
  modified_base (8),(10): m5c
gtggtggctcaagtatta

SEQ ID NO: 119 - DNA, 18 bp, Artificial sequence
  Synthetic oligonucleotide
  modified_base (1),(18): m5c
caagttggtttgtggtac

SEQ ID NO: 120 - DNA, 18 bp, Artificial sequence
  Synthetic oligonucleotide
  modified_base (2): m5c
gcaagttggtttgtggta

SEQ ID NO: 121 - DNA, 18 bp, Artificial sequence
  Synthetic oligonucleotide
  modified_base (3): m5c
tgcaagttggtttgtggt

SEQ ID NO: 122 - DNA, 18 bp, Artificial sequence
  Synthetic oligonucleotide
  modified_base (1),(4): m5c
ctgcaagttggtttgtgg

SEQ ID NO: 123 - DNA, 18 bp, Artificial sequence
  Synthetic oligonucleotide
  modified_base (1),(2),(5): m5c
cctgcaagttggtttgtg

SEQ ID NO: 124 - DNA, 18 bp, Artificial sequence
  Synthetic oligonucleotide
  modified_base (2),(3),(6): m5c
tcctgcaagttggtttgt

SEQ ID NO: 125 - DNA, 18 bp, Artificial sequence
  Synthetic oligonucleotide
  modified_base (2),(7): m5c
tctaggcaattgtggtgg

SEQ ID NO: 126 - DNA, 18 bp, Artificial sequence
  Synthetic oligonucleotide
  modified_base (2),(7),(16),(18): m5c
gcatggctaatgatgcac

SEQ ID NO: 127 - DNA, 18 bp, Artificial sequence
  Synthetic oligonucleotide
  modified_base (12),(16): m5c
tgtgaaggtagcgaacat

SEQ ID NO: 128 - DNA, 18 bp, Artificial sequence
  Synthetic oligonucleotide
  modified_base (13),(17): m5c
gtgtgaaggtagcgaaca

SEQ ID NO: 129 - DNA, 18 bp, Artificial sequence
  Synthetic oligonucleotide
  modified_base (5),(7),(10),(12),(15),(16),(17): m5c
gtaactctgcacttccca

SEQ ID NO: 130 - DNA, 18 bp, Artificial sequence
  Synthetic oligonucleotide
  modified_base (7),(9),(12),(14),(17),(18): m5c
aagtaactctgcacttcc

SEQ ID NO: 131 - DNA, 18 bp, Artificial sequence
  Synthetic oligonucleotide
  modified_base (3),(6),(7),(8),(14): m5c
gtcatccctatgtcttat

SEQ ID NO: 132 - DNA, 18 bp, Artificial sequence
  Synthetic oligonucleotide
  modified_base (2),(5),(9),(16),(18): m5c
gcaacagtctggattctc

SEQ ID NO: 133 - DNA, 18 bp, Artificial sequence
  Synthetic oligonucleotide
  modified_base (8),(9),(16): m5c
gaggtgtccttgttactg

SEQ ID NO: 134 - DNA, 18 bp, Artificial sequence
  Synthetic oligonucleotide
  modified_base (9),(10),(17): m5c
ggaggtgtccttgttact

SEQ ID NO: 135 - DNA, 18 bp, Artificial sequence
  Synthetic oligonucleotide
  modified_base (10),(11),(18): m5c
tggaggtgtccttgttac

SEQ ID NO: 136 - DNA, 18 bp, Artificial sequence
  Synthetic oligonucleotide
  modified_base (11),(12): m5c
gtggaggtgtccttgtta

SEQ ID NO: 137 - DNA, 18 bp, Artificial sequence
  Synthetic oligonucleotide
  modified_base (14),(15): m5c
attgtggaggtgtccttg

SEQ ID NO: 138 - DNA, 18 bp, Artificial sequence
  Synthetic oligonucleotide
  modified_base (1),(15),(16): m5c
cattgtggaggtgtcctt

SEQ ID NO: 139 - DNA, 18 bp, Artificial sequence
  Synthetic oligonucleotide
  modified_base (3),(17),(18): m5c
gacattgtggaggtgtcc

SEQ ID NO: 140 - DNA, 18 bp, Artificial sequence
  Synthetic oligonucleotide
  modified_base (4),(18): m5c
ggacattgtggaggtgtc

SEQ ID NO: 141 - DNA, 18 bp, Artificial sequence
  Synthetic oligonucleotide
  modified_base (1),(5): m5c
cggacattgtggaggtgt

SEQ ID NO: 142 - DNA, 18 bp, Artificial sequence
  Synthetic oligonucleotide
  modified_base (2),(6): m5c
acggacattgtggaggtg

SEQ ID NO: 143 - DNA, 18 bp, Artificial sequence
  Synthetic oligonucleotide
  modified_base (1),(3),(7): m5c
cacggacattgtggaggt

SEQ ID NO: 144 - DNA, 18 bp, Artificial sequence
  Synthetic oligonucleotide
  modified_base (1),(2),(4),(8): m5c
ccacggacattgtggagg

SEQ ID NO: 145 - DNA, 18 bp, Artificial sequence
  Synthetic oligonucleotide
  modified_base (1),(2),(4),(5),(7),(11): m5c
cctccacggacattgtgg

SEQ ID NO: 146 - DNA, 18 bp, Artificial sequence
  Synthetic oligonucleotide
  modified_base (3),(4),(6),(7),(9),(13): m5c
ggcctccacggacattgt

SEQ ID NO: 147 - DNA, 18 bp, Artificial sequence
  Synthetic oligonucleotide
  modified_base (4),(5),(7),(8),(10),(14): m5c
tggcctccacggacattg

SEQ ID NO: 148 - DNA, 18 bp, Artificial sequence
  Synthetic oligonucleotide
  modified_base (3),(11): m5c
gtcatatggtcagggtat

SEQ ID NO: 149 - DNA, 18 bp, Artificial sequence
  Synthetic oligonucleotide
  modified_base (4),(12): m5c
tgtcatatggtcagggta

SEQ ID NO: 150 - DNA, 18 bp, Artificial sequence
  Synthetic oligonucleotide
  modified_base (5),(13): m5c
atgtcatatggtcagggt

SEQ ID NO: 151 - DNA, 18 bp, Artificial sequence
  Synthetic oligonucleotide
  modified_base (6),(14): m5c
tatgtcatatggtcaggg

SEQ ID NO: 152 - DNA, 18 bp, Artificial sequence
  Synthetic oligonucleotide
  modified_base (3),(4),(5): m5c
tgcccaggagtatagatg

SEQ ID NO: 153 - DNA, 18 bp, Artificial sequence
  Synthetic oligonucleotide
  modified_base (3),(6),(8),(12): m5c
tacagcacttacggagtg

SEQ ID NO: 154 - DNA, 18 bp, Artificial sequence
  Synthetic oligonucleotide
  modified_base (4),(7),(9),(13): m5c
ttacagcacttacggagt

SEQ ID NO: 155 - DNA, 18 bp, Artificial sequence
  Synthetic oligonucleotide
  modified_base (2),(13),(16): m5c
gctatggatgtactacag

SEQ ID NO: 156 - DNA, 18 bp, Artificial sequence
  Synthetic oligonucleotide
  modified_base (5),(6),(7),(15): m5c
aagaccctttgaggcttt

SEQ ID NO: 157 - DNA, 18 bp, Artificial sequence
  Synthetic oligonucleotide
  modified_base (6),(7),(8),(16): m5c
taagaccctttgaggctt

SEQ ID NO: 158 - DNA, 18 bp, Artificial sequence
  Synthetic oligonucleotide
  modified_base (5),(7),(12),(14),(18): m5c
gtagctcttggcactagc

SEQ ID NO: 159 - DNA, 16 bp, Artificial sequence
  Synthetic oligonucleotide
  modified_base (2),(3),(14): m5c
tccgagatgttttcta

SEQ ID NO: 160 - DNA, 16 bp, Artificial sequence
  Synthetic oligonucleotide
  modified_base (2): m5c
tcaaaagtttccgaga

SEQ ID NO: 161 - DNA, 16 bp, Artificial sequence
  Synthetic oligonucleotide
  modified_base (1): m5c
caactatacgactgag

SEQ ID NO: 162 - DNA, 16 bp, Artificial sequence
  Synthetic oligonucleotide
  modified_base (2): m5c
tcaggaagtagtgtgg

SEQ ID NO: 163 - DNA, 16 bp, Artificial sequence
  Synthetic oligonucleotide
  modified_base (3): m5c
ttcgggtaagtagatt

SEQ ID NO: 164 - DNA, 16 bp, Artificial sequence
  Synthetic oligonucleotide
  modified_base (2): m5c
gcactatctgccaggg

SEQ ID NO: 165 - DNA, 16 bp, Artificial sequence
  Synthetic oligonucleotide
  modified_base (3),(14): m5c
gtcaatctagcagcat

SEQ ID NO: 166 - DNA, 16 bp, Artificial sequence
  Synthetic oligonucleotide
  modified_base (1),(16): m5c
cttcattgtgttgggc

SEQ ID NO: 167 - DNA, 16 bp, Artificial sequence
  Synthetic oligonucleotide
  modified_base (14),(15): m5c
tatgattttaggccca

SEQ ID NO: 168 - DNA, 16 bp, Artificial sequence
  Synthetic oligonucleotide
  modified_base (2),(16): m5c
tcagtttggagtttac

SEQ ID NO: 169 - DNA, 16 bp, Artificial sequence
  Synthetic oligonucleotide
  modified_base (14),(16): m5c
gatttgtgtgctcctc

SEQ ID NO: 170 - DNA, 16 bp, Artificial sequence
  Synthetic oligonucleotide
  modified_base (2),(15),(16): m5c
gctttcccatgctacc

SEQ ID NO: 171 - DNA, 16 bp, Artificial sequence
  Synthetic oligonucleotide
  modified_base (2),(14): m5c
gctcactcctggacaa

SEQ ID NO: 172 - DNA, 16 bp, Artificial sequence
  Synthetic oligonucleotide
  modified_base (2),(16): m5c
acgtgcgataatcttc

SEQ ID NO: 173 - DNA, 16 bp, Artificial sequence
  Synthetic oligonucleotide
agaaatgtaagccggg

SEQ ID NO: 174 - DNA, 16 bp, Artificial sequence
  Synthetic oligonucleotide
  modified_base (3): m5c
gtcattagcgtgcata

SEQ ID NO: 175 - DNA, 16 bp, Artificial sequence
  Synthetic oligonucleotide
  modified_base (15): m5c
tgggatgtaagcaaca

SEQ ID NO: 176 - DNA, 16 bp, Artificial sequence
  Synthetic oligonucleotide
  modified_base (3),(14): m5c
gactattgaaaggctg

SEQ ID NO: 177 - DNA, 16 bp, Artificial sequence
  Synthetic oligonucleotide
atgccccactctaata

SEQ ID NO: 178 - DNA, 16 bp, Artificial sequence
  Synthetic oligonucleotide
  modified_base (2),(14),(16): m5c
tctggatacaactcac

SEQ ID NO: 179 - DNA, 16 bp, Artificial sequence
  Synthetic oligonucleotide
agataggtcgctcagg

SEQ ID NO: 180 - DNA, 16 bp, Artificial sequence
  Synthetic oligonucleotide
  modified_base (2),(15): m5c
gcagagataggtcgct

SEQ ID NO: 181 - DNA, 16 bp, Artificial sequence
  Synthetic oligonucleotide
  modified_base (1),(3): m5c
cacggtaaagcactag

SEQ ID NO: 182 - DNA, 16 bp, Artificial sequence
  Synthetic oligonucleotide
  modified_base (1): m5c
cagtggcacggtaaag

SEQ ID NO: 183 - DNA, 16 bp, Artificial sequence
  Synthetic oligonucleotide
  modified_base (14): m5c
gaaacgccaagtgctg

SEQ ID NO: 184 - DNA, 16 bp, Artificial sequence
  Synthetic oligonucleotide
  modified_base (16): m5c
taagttctccctgggc

SEQ ID NO: 185 - DNA, 16 bp, Artificial sequence
  Synthetic oligonucleotide
  modified_base (14): m5c
atgaacgtctctgcag

SEQ ID NO: 186 - DNA, 16 bp, Artificial sequence
  Synthetic oligonucleotide
ttgacactatttcagg

SEQ ID NO: 187 - DNA, 16 bp, Artificial sequence
  Synthetic oligonucleotide
  modified_base (16): m5c
atagcttgctcaagac

SEQ ID NO: 188 - DNA, 16 bp, Artificial sequence
  Synthetic oligonucleotide
  modified_base (2),(14): m5c
gctgcatgtatcacta

SEQ ID NO: 189 - DNA, 16 bp, Artificial sequence
  Synthetic oligonucleotide
  modified_base (2),(14): m5c
gctaagtaggtgactt

SEQ ID NO: 190 - DNA, 16 bp, Artificial sequence
  Synthetic oligonucleotide
ttaggatgaagctaag

SEQ ID NO: 191 - DNA, 16 bp, Artificial sequence
  Synthetic oligonucleotide
  modified_base (1): m5c
ctgcactcggccctaa

SEQ ID NO: 192 - DNA, 16 bp, Artificial sequence
  Synthetic oligonucleotide
agattccaattgtgag

SEQ ID NO: 193 - DNA, 16 bp, Artificial sequence
  Synthetic oligonucleotide
  modified_base (3),(16): m5c
agcctatcaccacgtc

SEQ ID NO: 194 - DNA, 16 bp, Artificial sequence
  Synthetic oligonucleotide
  modified_base (1),(16): m5c
cagcgtcacccaaatc

SEQ ID NO: 195 - DNA, 16 bp, Artificial sequence
  Synthetic oligonucleotide
  modified_base (3),(16): m5c
tacttagaagggctgc

SEQ ID NO: 196 - DNA, 16 bp, Artificial sequence
  Synthetic oligonucleotide
  modified_base (2),(3): m5c
gcctagtcactttgat

SEQ ID NO: 197 - DNA, 16 bp, Artificial sequence
  Synthetic oligonucleotide
  modified_base (2),(14): m5c
tcagggtagatgtcaa

SEQ ID NO: 198 - DNA, 16 bp, Artificial sequence
  Synthetic oligonucleotide
taggtgttcagggtag

SEQ ID NO: 199 - DNA, 16 bp, Artificial sequence
  Synthetic oligonucleotide
agtcaaagctaggtgt

SEQ ID NO: 200 - DNA, 16 bp, Artificial sequence
  Synthetic oligonucleotide
  modified_base (14),(15),(16): m5c
aatggatactctgccc

SEQ ID NO: 201 - DNA, 16 bp, Artificial sequence
  Synthetic oligonucleotide
  modified_base (2),(3),(16): m5c
tccccaagctagatgc

SEQ ID NO: 202 - DNA, 16 bp, Artificial sequence
  Synthetic oligonucleotide
  modified_base (2),(16): m5c
acgtgtggtttgcatc

SEQ ID NO: 203 - DNA, 16 bp, Artificial sequence
  Synthetic oligonucleotide
  modified_base (3): m5c
gtcaaacgtgtggttt

SEQ ID NO: 204 - DNA, 16 bp, Artificial sequence
  Synthetic oligonucleotide
aggtgtcaaacgtgtg

SEQ ID NO: 205 - DNA, 16 bp, Artificial sequence
  Synthetic oligonucleotide
  modified_base (1),(14): m5c
ctatttaaggtgtcaa

SEQ ID NO: 206 - DNA, 16 bp, Artificial sequence
  Synthetic oligonucleotide
  modified_base (3),(14): m5c
atcagactgcctgcat

SEQ ID NO: 207 - DNA, 16 bp, Artificial sequence
  Synthetic oligonucleotide
  modified_base (2): m5c
gcacttacaaggctgg

SEQ ID NO: 208 - DNA, 16 bp, Artificial sequence
  Synthetic oligonucleotide
  modified_base (16): m5c
ggtgctgctaatatac

SEQ ID NO: 209 - DNA, 16 bp, Artificial sequence
  Synthetic oligonucleotide
  modified_base (2),(14): m5c
gcactaataagcacta

SEQ ID NO: 210 - DNA, 16 bp, Artificial sequence
  Synthetic oligonucleotide
  modified_base (2),(16): m5c
tcatgcagcctgttac

SEQ ID NO: 211 - DNA, 16 bp, Artificial sequence
  Synthetic oligonucleotide
  modified_base (16): m5c
aagcactagttattgc

SEQ ID NO: 212 - DNA, 16 bp, Artificial sequence
  Synthetic oligonucleotide
  modified_base (3): m5c
tgcctgaccctgttta

SEQ ID NO: 213 - DNA, 16 bp, Artificial sequence
  Synthetic oligonucleotide
  modified_base (3): m5c
agcttgataaccttag

SEQ ID NO: 214 - DNA, 16 bp, Artificial sequence
  Synthetic oligonucleotide
gatgtagtagagtttt

SEQ ID NO: 215 - DNA, 16 bp, Artificial sequence
  Synthetic oligonucleotide
  modified_base (3): m5c
agctgatgtagtagag

SEQ ID NO: 216 - DNA, 16 bp, Artificial sequence
  Synthetic oligonucleotide
  modified_base (15): m5c
gttggtttgtggtact

SEQ ID NO: 217 - DNA, 16 bp, Artificial sequence
  Synthetic oligonucleotide
  modified_base (16): m5c
gtaggattctggttac

SEQ ID NO: 218 - DNA, 16 bp, Artificial sequence
  Synthetic oligonucleotide
  modified_base (16): m5c
ataagtacctttgatc

SEQ ID NO: 219 - DNA, 16 bp, Artificial sequence
  Synthetic oligonucleotide
gaaggtagcgaacatg

SEQ ID NO: 220 - DNA, 16 bp, Artificial sequence
  Synthetic oligonucleotide
ggtaactgctccttaa

SEQ ID NO: 221 - DNA, 16 bp, Artificial sequence
  Synthetic oligonucleotide
  modified_base (15),(16): m5c
gtaactctgcacttcc

SEQ ID NO: 222 - DNA, 16 bp, Artificial sequence
  Synthetic oligonucleotide
  modified_base (14),(16): m5c
gaaagtaactctgcac

SEQ ID NO: 223 - DNA, 16 bp, Artificial sequence
  Synthetic oligonucleotide
  modified_base (1): m5c
cgagacctggaaagta

SEQ ID NO: 224 - DNA, 16 bp, Artificial sequence
  Synthetic oligonucleotide
  modified_base (3),(14): m5c
gtcatccctatgtctt

SEQ ID NO: 225 - DNA, 16 bp, Artificial sequence
  Synthetic oligonucleotide
  modified_base (15): m5c
gtgttttggctgtact

SEQ ID NO: 226 - DNA, 16 bp, Artificial sequence
  Synthetic oligonucleotide
  modified_base (16): m5c
agtctggattctctac

SEQ ID NO: 227 - DNA, 16 bp, Artificial sequence
  Synthetic oligonucleotide
atatggtcagggtatg

SEQ ID NO: 228 - DNA, 16 bp, Artificial sequence
  Synthetic oligonucleotide
gagtatagatgctatg

SEQ ID NO: 229 - DNA, 16 bp, Artificial sequence
  Synthetic oligonucleotide
  modified_base (15): m5c
atgctatggatgtact

SEQ ID NO: 230 - DNA, 16 bp, Artificial sequence
  Synthetic oligonucleotide
gagtattacatgctat

SEQ ID NO: 231 - DNA, 16 bp, Artificial sequence
  Synthetic oligonucleotide
  modified_base (15): m5c
tttctatttgagcacg

SEQ ID NO: 232 - DNA, 16 bp, Artificial sequence
  Synthetic oligonucleotide
gtatacagttgaaggg

SEQ ID NO: 233 - DNA, 16 bp, Artificial sequence
  Synthetic oligonucleotide
  modified_base (2): m5c
gctgtaaggttttgat

SEQ ID NO: 234 - DNA, 16 bp, Artificial sequence
  Synthetic oligonucleotide
  modified_base (14): m5c
ggagacttgcctgcat

SEQ ID NO: 235 - DNA, 16 bp, Artificial sequence
  Synthetic oligonucleotide
  modified_base (16): m5c
gtacgtatgtttagtc

SEQ ID NO: 236 - DNA, 16 bp, Artificial sequence
  Synthetic oligonucleotide
  modified_base (2): m5c
tcatggtgggtacgta

SEQ ID NO: 237 - DNA, 16 bp, Artificial sequence
  Synthetic oligonucleotide
  modified_base (16): m5c
gtgtaagggaaacttc

SEQ ID NO: 238 - DNA, 16 bp, Artificial sequence
  Synthetic oligonucleotide
  modified_base (1),(16): m5c
cttgagggagtagtac

SEQ ID NO: 239 - DNA, 18 bp, Artificial sequence
  Synthetic oligonucleotide
tcgggtaagtagattttc

SEQ ID NO: 240 - DNA, 18 bp, Artificial sequence
  Synthetic oligonucleotide
gaagtatctgtaggccta

SEQ ID NO: 241 - DNA, 18 bp, Artificial sequence
  Synthetic oligonucleotide
ggactgtataggagatta

SEQ ID NO: 242 - DNA, 18 bp, Artificial sequence
  Synthetic oligonucleotide
ggttataggatgcaggta

SEQ ID NO: 243 - DNA, 18 bp, Artificial sequence
  Synthetic oligonucleotide
aggttataggatgcaggt

SEQ ID NO: 244 - DNA, 18 bp, Artificial sequence
  Synthetic oligonucleotide
gaagctaagtaggtgact

SEQ ID NO: 245 - DNA, 18 bp, Artificial sequence
  Synthetic oligonucleotide
tgaagctaagtaggtgac

SEQ ID NO: 246 - DNA, 18 bp, Artificial sequence
  Synthetic oligonucleotide
cctagtcactttgataga

SEQ ID NO: 247 - DNA, 18 bp, Artificial sequence
  Synthetic oligonucleotide
ggaacatcttgagtaggt

SEQ ID NO: 248 - DNA, 18 bp, Artificial sequence
  Synthetic oligonucleotide
ggtgttcagggtagatgt

SEQ ID NO: 249 - DNA, 18 bp, Artificial sequence
  Synthetic oligonucleotide
ggatactctgccctgttc

SEQ ID NO: 250 - DNA, 18 bp, Artificial sequence
  Synthetic oligonucleotide
ggtgtcaaacgtgtggtt

SEQ ID NO: 251 - DNA, 18 bp, Artificial sequence
  Synthetic oligonucleotide
ccgtgtgctagtatttgt

SEQ ID NO: 252 - DNA, 18 bp, Artificial sequence
  Synthetic oligonucleotide
tagtagagttttgcttgg

SEQ ID NO: 253 - DNA, 18 bp, Artificial sequence
  Synthetic oligonucleotide
gatgtagtagagttttgc

SEQ ID NO: 254 - DNA, 18 bp, Artificial sequence
  Synthetic oligonucleotide
tgatgtagtagagttttg

SEQ ID NO: 255 - DNA, 18 bp, Artificial sequence
  Synthetic oligonucleotide
ctgatgtagtagagtttt

SEQ ID NO: 256 - DNA, 18 bp, Artificial sequence
  Synthetic oligonucleotide
gcaagttggtttgtggta

SEQ ID NO: 257 - DNA, 18 bp, Artificial sequence
  Synthetic oligonucleotide
tctaggcaattgtggtgg

SEQ ID NO: 258 - DNA, 18 bp, Artificial sequence
  Synthetic oligonucleotide
gtaactctgcacttccca

SEQ ID NO: 259 - DNA, 18 bp, Artificial sequence
  Synthetic oligonucleotide
gtcatccctatgtcttat

SEQ ID NO: 260 - DNA, 18 bp, Artificial sequence
  Synthetic oligonucleotide
gtcatatggtcagggtat

SEQ ID NO: 261 - DNA, 18 bp, Artificial sequence
  Synthetic oligonucleotide
tgtcatatggtcagggta

SEQ ID NO: 262 - DNA, 18 bp, Artificial sequence
  Synthetic oligonucleotide
atgtcatatggtcagggt

SEQ ID NO: 263 - DNA, 18 bp, Artificial sequence
  Synthetic oligonucleotide
tatgtcatatggtcaggg

SEQ ID NO: 264 - DNA, 16 bp, Artificial sequence
  Synthetic oligonucleotide
tcagtttggagtttac

SEQ ID NO: 265 - DNA, 16 bp, Artificial sequence
  Synthetic oligonucleotide
taagttctccctgggc

SEQ ID NO: 266 - DNA, 16 bp, Artificial sequence
  Synthetic oligonucleotide
atagcttgctcaagac

SEQ ID NO: 267 - DNA, 16 bp, Artificial sequence
  Synthetic oligonucleotide
cagcgtcacccaaatc

SEQ ID NO: 268 - DNA, 16 bp, Artificial sequence
  Synthetic oligonucleotide
gtcaaacgtgtggttt

SEQ ID NO: 269 - DNA, 16 bp, Artificial sequence
  Synthetic oligonucleotide
ggtgctgctaatatac

SEQ ID NO: 270 - DNA, 16 bp, Artificial sequence
  Synthetic oligonucleotide
gtcatccctatgtctt

SEQ ID NO: 271 - DNA, 16 bp, Artificial sequence
  Synthetic oligonucleotide
gtgttttggctgtact

SEQ ID NO: 272 - DNA, 18 bp, Artificial Sequence
  Synthetic oligonucleotide
  modified_base (9),(11),(13): m5c
agataggtcgctcaggag

SEQ ID NO: 273 - DNA, 18 bp, Artificial Sequence
  Synthetic oligonucleotide
  modified_base (10),(12),(14): m5c
gagataggtcgctcagga

SEQ ID NO: 274 - DNA, 18 bp, Artificial Sequence
  Synthetic oligonucleotide
  modified_base (11),(13),(15): m5c
agagataggtcgctcagg

SEQ ID NO: 275 - DNA, 18 bp, Artificial Sequence
  Synthetic oligonucleotide
  modified_base (9): m5c
taggtgttcagggtagat

SEQ ID NO: 276 - DNA, 18 bp, Artificial Sequence
  Synthetic oligonucleotide
  modified_base (1),(10): m5c
ctaggtgttcagggtaga

SEQ ID NO: 277 - DNA, 18 bp, Artificial Sequence
  Synthetic oligonucleotide
  modified_base (2),(13),(16),(17),(18): m5c
acgtgtggtttgcatccc

SEQ ID NO: 278 - DNA, 18 bp, Artificial Sequence
  Synthetic oligonucleotide
  modified_base (3),(14),(17),(18): m5c
aacgtgtggtttgcatcc

SEQ ID NO: 279 - DNA, 18 bp, Artificial Sequence
  Synthetic oligonucleotide
  modified_base (4),(15),(18): m5c
aaacgtgtggtttgcatc

SEQ ID NO: 280 - DNA, 18 bp, Artificial Sequence
  Synthetic oligonucleotide
  modified_base (5),(9): m5c
gtgtcaaacgtgtggttt

SEQ ID NO: 281 - DNA, 18 bp, Artificial Sequence
  Synthetic oligonucleotide
  modified_base (7),(11): m5c
aggtgtcaaacgtgtggt

SEQ ID NO: 282 - DNA, 18 bp, Artificial Sequence
  Synthetic oligonucleotide
  modified_base (8),(12): m5c
aaggtgtcaaacgtgtgg

SEQ ID NO: 283 - DNA, 18 bp, Artificial Sequence
  Synthetic oligonucleotide
  modified_base (9),(13): m5c
taaggtgtcaaacgtgtg

SEQ ID NO: 284 - DNA, 18 bp, Artificial Sequence
  Synthetic oligonucleotide
  modified_base (17): m5c
aagttggtttgtggtact

SEQ ID NO: 285 - DNA, 18 bp, Artificial Sequence
  Synthetic oligonucleotide
  modified_base (6),(8),(11),(13),(16),(17),(18): m5c
agtaactctgcacttccc